European Patent Application EP 4 506 454 A1, published February 12, 2025. Title: 一种腺苷脱氨酶、碱基编辑器及应用. Applicant: 尧唐(上海)生物科技有限公司. The sequence listing filed with the application follows.

SEQUENCE LISTING (233 sequences)

SEQ ID NO: 1 - protein, 170 aa, synthetic construct
MSELNDAYWMKQALALAQKAREQGEVPVGAILVLDDEVIGQGWNRAITLHDPTAHAEIMALQQGGQIVQNYRLLNATLYVTFEPCVMCAGAMVHSRIKRLVYGVSNSKRGAAGSLLNVLNYPGMNHQIEITAGVMANECSEMLCQFYQQPREVFNAEREARRLNQPDRAD

SEQ ID NO: 2 - DNA, 510 bp, synthetic construct
  source 1..510: mol_type = other DNA
atgagtgagctgaatgatgcttactggatgaaacaggcactcgctttagctcagaaggcccgggaacagggagaagttccagtgggcgctattctggtgctggatgatgaagtgataggacagggatggaatagagccatcaccctgcacgaccccaccgcccacgccgagatcatggccctgcagcagggcggccagatcgtgcagaactaccggctgctgaacgccaccctgtacgtgaccttcgagccctgcgtgatgtgcgccggcgccatggtgcacagcaggatcaagagactggtctacggcgtgagcaactcaaaaagaggcgccgccggcagcctgctgaacgtgctgaactaccccggcatgaaccaccagatcgagatcaccgccggcgtgatggccaacgagtgcagcgagatgctgtgccagttctatcagcagcctagggaagtgttcaatgctgagcgtgaggctaggcggctgaaccaacctgatagagctgac

SEQ ID NO: 3 - protein, 1609 aa, synthetic construct
MKRTADGSEFESPKKKRKVMSELNDAYWMKQALALAQKAREQGEVPVGAILVLDDEVIGQGWNRAITLHDPTAHAEIMALQQGGQIVQNYRLLNATLYVTFEPCVMCAGAMVHSRIKRLVYGVSNSKRGAAGSLLNVLNYPGMNHQIEITAGVMANECSEMLCQFYQQPREVFNAEREARRLNQPDRADSGGSSGGSSGSETPGTSESATPESSGGSSGGSDKKYSIGLAIGTNSVGWAVITDEYKVPSKKFKVLGNTDRHSIKKNLIGALLFDSGETAEATRLKRTARRRYTRRKNRICYLQEIFSNEMAKVDDSFFHRLEESFLVEEDKKHERHPIFGNIVDEVAYHEKYPTIYHLRKKLVDSTDKADLRLIYLALAHMIKFRGHFLIEGDLNPDNSDVDKLFIQLVQTYNQLFEENPINASGVDAKAILSARLSKSRRLENLIAQLPGEKKNGLFGNLIALSLGLTPNFKSNFDLAEDAKLQLSKDTYDDDLDNLLAQIGDQYADLFLAAKNLSDAILLSDILRVNTEITKAPLSASMIKRYDEHHQDLTLLKALVRQQLPEKYKEIFFDQSKNGYAGYIDGGASQEEFYKFIKPILEKMDGTEELLVKLNREDLLRKQRTFDNGSIPHQIHLGELHAILRRQEDFYPFLKDNREKIEKILTFRIPYYVGPLARGNSRFAWMTRKSEETITPWNFEEVVDKGASAQSFIERMTNFDKNLPNEKVLPKHSLLYEYFTVYNELTKVKYVTEGMRKPAFLSGEQKKAIVDLLFKTNRKVTVKQLKEDYFKKIECFDSVEISGVEDRFNASLGTYHDLLKIIKDKDFLDNEENEDILEDIVLTLTLFEDREMIEERLKTYAHLFDDKVMKQLKRRRYTGWGRLSRKLINGIRDKQSGKTILDFLKSDGFANRNFMQLIHDDSLTFKEDIQKAQVSGQGDSLHEHIANLAGSPAIKKGILQTVKVVDELVKVMGRHKPENIVIEMARENQTTQKGQKNSRERMKRIEEGIKELGSQILKEHPVENTQLQNEKLYLYYLQNGRDMYVDQELDINRLSDYDVDHIVPQSFLKDDSIDNKVLTRSDKNRGKSDNVPSEEVVKKMKNYWRQLLNAKLITQRKFDNLTKAERGGLSELDKAGFIKRQLVETRQITKHVAQILDSRMNTKYDENDKLIREVKVITLKSKLVSDFRKDFQFYKVREINNYHHAHDAYLNAVVGTALIKKYPKLESEFVYGDYKVYDVRKMIAKSEQEIGKATAKYFFYSNIMNFFKTEITLANGEIRKRPLIETNGETGEIVWDKGRDFATVRKVLSMPQVNIVKKTEVQTGGFSKESILPKRNSDKLIARKKDWDPKKYGGFDSPTVAYSVLVVAKVEKGKSKKLKSVKELLGITIMERSSFEKNPIDFLEAKGYKEVKKDLIIKLPKYSLFELENGRKRMLASAGELQKGNELALPSKYVNFLYLASHYEKLKGSPEDNEQKQLFVEQHKHYLDEIIEQISEFSKRVILADANLDKVLSAYNKHRDKPIREQAENIIHLFTLTNLGAPAAFKYFDTTIDRKRYTSTKEVLDATLIHQSITGLYETRIDLSQLGGDSGGSKRTADGSEFEPKKKRKV

SEQ ID NO: 4 - DNA, 4827 bp, synthetic construct
  source 1..4827: mol_type = other DNA
atgaaacggacagccgacggaagcgagttcgagtcaccaaagaagaagcggaaagtcatgagtgagctgaatgatgcttactggatgaaacaggcactcgctttagctcagaaggcccgggaacagggagaagttccagtgggcgctattctggtgctggatgatgaagtgataggacagggatggaatagagccatcaccctgcacgaccccaccgcccacgccgagatcatggccctgcagcagggcggccagatcgtgcagaactaccggctgctgaacgccaccctgtacgtgaccttcgagccctgcgtgatgtgcgccggcgccatggtgcacagcaggatcaagagactggtctacggcgtgagcaactcaaaaagaggcgccgccggcagcctgctgaacgtgctgaactaccccggcatgaaccaccagatcgagatcaccgccggcgtgatggccaacgagtgcagcgagatgctgtgccagttctatcagcagcctagggaagtgttcaatgctgagcgtgaggctaggcggctgaaccaacctgatagagctgactccggaggatctagcggaggctcctctggctctgagacacctggcacaagcgagagcgcaacacctgaaagcagcgggggcagcagcggggggtcagacaagaagtacagcatcggcctggccatcggcaccaactctgtgggctgggccgtgatcaccgacgagtacaaggtgcccagcaagaaattcaaggtgctgggcaacaccgaccggcacagcatcaagaagaacctgatcggagccctgctgttcgacagcggcgaaacagccgaggccacccggctgaagagaaccgccagaagaagatacaccagacggaagaaccggatctgctatctgcaagagatcttcagcaacgagatggccaaggtggacgacagcttcttccacagactggaagagtccttcctggtggaagaggataagaagcacgagcggcaccccatcttcggcaacatcgtggacgaggtggcctaccacgagaagtaccccaccatctaccacctgagaaagaaactggtggacagcaccgacaaggccgacctgcggctgatctatctggccctggcccacatgatcaagttccggggccacttcctgatcgagggcgacctgaaccccgacaacagcgacgtggacaagctgttcatccagctggtgcagacctacaaccagctgttcgaggaaaaccccatcaacgccagcggcgtggacgccaaggccatcctgtctgccagactgagcaagagcagacggctggaaaatctgatcgcccagctgcccggcgagaagaagaatggcctgttcggaaacctgattgccctgagcctgggcctgacccccaacttcaagagcaacttcgacctggccgaggatgccaaactgcagctgagcaaggacacctacgacgacgacctggacaacctgctggcccagatcggcgaccagtacgccgacctgtttctggccgccaagaacctgtccgacgccatcctgctgagcgacatcctgagagtgaacaccgagatcaccaaggcccccctgagcgcctctatgatcaagagatacgacgagcaccaccaggacctgaccctgctgaaagctctcgtgcggcagcagctgcctgagaagtacaaagagattttcttcgaccagagcaagaacggctacgccggctacattgacggcggagccagccaggaagagttctacaagttcatcaagcccatcctggaaaagatggacggcaccgaggaactgctcgtgaagctgaacagagaggacctgctgcggaagcagcggaccttcgacaacggcagcatcccccaccagatccacctgggagagctgcacgccattctgcggcggcaggaagatttttacccattcctgaaggacaaccgggaaaagatcgagaagatcctgaccttccgcatcccctactacgtgggccctctggccaggggaaacagcagattcgcctggatgaccagaaagagcgaggaaaccatcaccccctggaacttcgaggaagtggtggacaagggcgcttccgcccagagcttcatcgagcggatgaccaacttcgataagaacctgcccaacgagaaggtgctgcccaagcacagcctgctgtacgagtacttcaccgtgtataacgagctgaccaaagtgaaatacgtgaccgagggaatgagaaagcccgccttcctgagcggcgagcagaaaaaggccatcgtggacctgctgttcaagaccaaccggaaagtgaccgtgaagcagctgaaagaggactacttcaagaaaatcgagtgcttcgactccgtggaaatctccggcgtggaagatcggttcaacgcctccctgggcacataccacgatctgctgaaaattatcaaggacaaggacttcctggacaatgaggaaaacgaggacattctggaagatatcgtgctgaccctgacactgtttgaggacagagagatgatcgaggaacggctgaaaacctatgcccacctgttcgacgacaaagtgatgaagcagctgaagcggcggagatacaccggctggggcaggctgagccggaagctgatcaacggcatccgggacaagcagtccggcaagacaatcctggatttcctgaagtccgacggcttcgccaacagaaacttcatgcagctgatccacgacgacagcctgacctttaaagaggacatccagaaagcccaggtgtccggccagggcgatagcctgcacgagcacattgccaatctggccggcagccccgccattaagaagggcatcctgcagacagtgaaggtggtggacgagctcgtgaaagtgatgggccggcacaagcccgagaacatcgtgatcgaaatggccagagagaaccagaccacccagaagggacagaagaacagccgcgagagaatgaagcggatcgaagagggcatcaaagagctgggcagccagatcctgaaagaacaccccgtggaaaacacccagctgcagaacgagaagctgtacctgtactacctgcagaatgggcgggatatgtacgtggaccaggaactggacatcaaccggctgtccgactacgatgtggaccatatcgtgcctcagagctttctgaaggacgactccatcgacaacaaggtgctgaccagaagcgacaagaaccggggcaagagcgacaacgtgccctccgaagaggtcgtgaagaagatgaagaactactggcggcagctgctgaacgccaagctgattacccagagaaagttcgacaatctgaccaaggccgagagaggcggcctgagcgaactggataaggccggcttcatcaagagacagctggtggaaacccggcagatcacaaagcacgtggcacagatcctggactcccggatgaacactaagtacgacgagaatgacaagctgatccgggaagtgaaagtgatcaccctgaagtccaagctggtgtccgatttccggaaggatttccagttttacaaagtgcgcgagatcaacaactaccaccacgcccacgacgcctacctgaacgccgtcgtgggaaccgccctgatcaaaaagtaccctaagctggaaagcgagttcgtgtacggcgactacaaggtgtacgacgtgcggaagatgatcgccaagagcgagcaggaaatcggcaaggctaccgccaagtacttcttctacagcaacatcatgaactttttcaagaccgagattaccctggccaacggcgagatccggaagcggcctctgatcgagacaaacggcgaaaccggggagatcgtgtgggataagggccgggattttgccaccgtgcggaaagtgctgagcatgccccaagtgaatatcgtgaaaaagaccgaggtgcagacaggcggcttcagcaaagagtctatcctgcccaagaggaacagcgataagctgatcgccagaaagaaggactgggaccctaagaagtacggcggcttcgacagccccaccgtggcctattctgtgctggtggtggccaaagtggaaaagggcaagtccaagaaactgaagagtgtgaaagagctgctggggatcaccatcatggaaagaagcagcttcgagaagaatcccatcgactttctggaagccaagggctacaaagaagtgaaaaaggacctgatcatcaagctgcctaagtactccctgttcgagctggaaaacggccggaagagaatgctggcctctgccggcgaactgcagaagggaaacgaactggccctgccctccaaatatgtgaacttcctgtacctggccagccactatgagaagctgaagggctcccccgaggataatgagcagaaacagctgtttgtggaacagcacaagcactacctggacgagatcatcgagcagatcagcgagttctccaagagagtgatcctggccgacgctaatctggacaaagtgctgtccgcctacaacaagcaccgggataagcccatcagagagcaggccgagaatatcatccacctgtttaccctgaccaatctgggagcccctgccgccttcaagtactttgacaccaccatcgaccggaagaggtacaccagcaccaaagaggtgctggacgccaccctgatccaccagagcatcaccggcctgtacgagacacggatcgacctgtctcagctgggaggtgactctggcggctcaaaaagaaccgccgacggcagcgaattcgagcccaagaagaagaggaaagtc

SEQ ID NO: 5 - DNA, 57 bp, synthetic construct
  source 1..57: mol_type = other DNA
ggctacggtctcatgccagttctatggtatgcgcagagaagtgttcaatgctgagcg

SEQ ID NO: 6 - DNA, 33 bp, synthetic construct
  source 1..33: mol_type = other DNA
ggctacggtctcaggcacagcatctcgctgcac

SEQ ID NO: 7 - DNA, 57 bp, synthetic construct
  source 1..57: mol_type = other DNA
ggctacggtctcacagcagcctaggaggccacatactgctgagcgtgaggctaggcg

SEQ ID NO: 8 - DNA, 33 bp, synthetic construct
  source 1..33: mol_type = other DNA
ggctacggtctcagctgatagaactggcacagc

SEQ ID NO: 9 - DNA, 57 bp, synthetic construct
  source 1..57: mol_type = other DNA
ggctacggtctcatgccagttctatccgggtcttcgcgaagtgttcaatgctgagcg

SEQ ID NO: 10 - DNA, 33 bp, synthetic construct; identical to SEQ ID NO: 6
  source 1..33: mol_type = other DNA

SEQ ID NO: 11 - DNA, 57 bp, synthetic construct
  source 1..57: mol_type = other DNA
ggctacggtctcacagcagcctaggacgttttttacggctgagcgtgaggctaggcg

SEQ ID NO: 12 - DNA, 33 bp, synthetic construct; identical to SEQ ID NO: 8
  source 1..33: mol_type = other DNA

SEQ ID NO: 13 - DNA, 49 bp, synthetic construct
  source 1..49: mol_type = other DNA
ggctacggtctcaggtctacggcgtgaggaactcaaaaagaggcgccgc

SEQ ID NO: 14 - DNA, 33 bp, synthetic construct
  source 1..33: mol_type = other DNA
ggctacggtctcagaccagtctcttgatcctgc

SEQ ID NO: 15 - DNA, 57 bp, synthetic construct
  source 1..57: mol_type = other DNA
ggctacggtctcacagcagcctagggggataaagcgcgctgagcgtgaggctaggcg

SEQ ID NO: 16 - DNA, 33 bp, synthetic construct; identical to SEQ ID NO: 8
  source 1..33: mol_type = other DNA

SEQ ID NO: 17 - DNA, 57 bp, synthetic construct
  source 1..57: mol_type = other DNA
ggctacggtctcatgccagttctattgcctccgaaaggaagtgttcaatgctgagcg

SEQ ID NO: 18 - DNA, 33 bp, synthetic construct; identical to SEQ ID NO: 6
  source 1..33: mol_type = other DNA

SEQ ID NO: 19 - DNA, 57 bp, synthetic construct
  source 1..57: mol_type = other DNA
ggctacggtctcacagcagcctaggtggacactgcacgctgagcgtgaggctaggcg

SEQ ID NO: 20 - DNA, 43 bp, synthetic construct
  source 1..43: mol_type = other DNA
ggctacggtctcagctgatagaactggcacagcatctcgctgc

SEQ ID NO: 21 - DNA, 49 bp, synthetic construct
  source 1..49: mol_type = other DNA
ggctacggtctcaggtctacggcgtgaaaaactcaaaaagaggcgccgc

SEQ ID NO: 22 - DNA, 44 bp, synthetic construct
  source 1..44: mol_type = other DNA
ggctacggtctcagaccagtctcttgatcctgctgtgcaccatg

SEQ ID NO: 23 - DNA, 52 bp, synthetic construct
  source 1..52: mol_type = other DNA
taggacagggatggaatagatgctacggccatcacgaccccaccgcccacgc

SEQ ID NO: 24 - DNA, 20 bp, synthetic construct
  source 1..20: mol_type = other DNA
tctattccatccctgtccta

SEQ ID NO: 25 - DNA, 49 bp, synthetic construct
  source 1..49: mol_type = other DNA
ggctacggtctcaggtctacggcgtggctaactcaaaaagaggcgccgc

SEQ ID NO: 26 - DNA, 44 bp, synthetic construct; identical to SEQ ID NO: 22
  source 1..44: mol_type = other DNA

SEQ ID NO: 27 - DNA, 52 bp, synthetic construct
  source 1..52: mol_type = other DNA
ggatcaagagactggtctacggcatgagcaactcaaaaagaggcgccgccgg

SEQ ID NO: 28 - DNA, 18 bp, synthetic construct
  source 1..18: mol_type = other DNA
gccgtagaccagtctctt

SEQ ID NO: 29 - DNA, 52 bp, synthetic construct
  source 1..52: mol_type = other DNA
ggatcaagagactggtctacggcgtgtgcaactcaaaaagaggcgccgccgg

SEQ ID NO: 30 - DNA, 30 bp, synthetic construct
  source 1..30: mol_type = other DNA
acgccgtagaccagtctcttgatcctgctg

SEQ ID NO: 31 - DNA, 57 bp, synthetic construct
  source 1..57: mol_type = other DNA
ggctacggtctcatgccagttctatgcagggtgtcgtgaagtgttcaatgctgagcg

SEQ ID NO: 32 - DNA, 33 bp, synthetic construct; identical to SEQ ID NO: 6
  source 1..33: mol_type = other DNA

SEQ ID NO: 33 - DNA, 40 bp, synthetic construct
  source 1..40: mol_type = other DNA
gatcaagagactggtctacgtgagcaactcaaaaagaggc

SEQ ID NO: 34 - DNA, 20 bp, synthetic construct
  source 1..20: mol_type = other DNA
cgtagaccagtctcttgatc

SEQ ID NO: 35 - DNA, 47 bp, synthetic construct
  source 1..47: mol_type = other DNA
acagggatggaatagagccagaggaacgcacgaccccaccgcccacg

SEQ ID NO: 36 - DNA, 20 bp, synthetic construct
  source 1..20: mol_type = other DNA
tctattccatccctgtccta

SEQ ID NO: 37 - DNA, 50 bp, synthetic construct
  source 1..50: mol_type = other DNA
ccagtgggcgctattctggtcttgggcaacgaagtgataggacagggatg

SEQ ID NO: 38 - DNA, 20 bp, synthetic construct
  source 1..20: mol_type = other DNA
cagaatagcgcccactggaa

SEQ ID NO: 39 - DNA, 51 bp, synthetic construct
  source 1..51: mol_type = other DNA
ctggatgaaacaggcactcgtttgcagggagacagggagaagttccagtgg

SEQ ID NO: 40 - DNA, 20 bp, synthetic construct
  source 1..20: mol_type = other DNA
cgagtgcctgtttcatccag

SEQ ID NO: 41 - DNA, 52 bp, synthetic construct
  source 1..52: mol_type = other DNA
ctggatgaaacaggcactcgcttgcggagactcagggagaagttccagtggg

SEQ ID NO: 42 - DNA, 20 bp, synthetic construct
  source 1..20: mol_type = other DNA
cgagtgcctgtttcatccag

SEQ ID NO: 43 - DNA, 52 bp, synthetic construct
  source 1..52: mol_type = other DNA
ctggatgaaacaggcactcgcgagcgactcgccagggagaagttccagtggg

SEQ ID NO: 44 - RNA, 20 nt, synthetic construct
  source 1..20: mol_type = other RNA
cgagtgcctgtttcatccag

SEQ ID NO: 45 - DNA, 49 bp, synthetic construct
  source 1..49: mol_type = other DNA
ctggatgaaacaggcactcgcacgcgtttgaacagggagaagttccagt

SEQ ID NO: 46 - DNA, 20 bp, synthetic construct
  source 1..20: mol_type = other DNA
cgagtgcctgtttcatccag

SEQ ID NO: 47 - DNA, 44 bp, synthetic construct
  source 1..44: mol_type = other DNA
aacaggcactcgaaggcccgtctccagggagaagttccagtggg

SEQ ID NO: 48 - DNA, 20 bp, synthetic construct
  source 1..20: mol_type = other DNA
cgagtgcctgtttcatccag

SEQ ID NO: 49 - DNA, 51 bp, synthetic construct
  source 1..51: mol_type = other DNA
ctggatgaaacaggcactcgctcgggttttcacagggagaagttccagtgg

SEQ ID NO: 50 - DNA, 20 bp, synthetic construct
  source 1..20: mol_type = other DNA
cgagtgcctgtttcatccag

SEQ ID NO: 51 - DNA, 52 bp, synthetic construct
  source 1..52: mol_type = other DNA
ctggatgaaacaggcactcgtacatcggatcccagggagaagttccagtggg

SEQ ID NO: 52 - DNA, 20 bp, synthetic construct
  source 1..20: mol_type = other DNA
cgagtgcctgtttcatccag

SEQ ID NO: 53 - DNA, 50 bp, synthetic construct
  source 1..50: mol_type = other DNA
ggatgaaacaggcactcgaaagcatttgaccagggagaagttccagtggg

SEQ ID NO: 54 - DNA, 20 bp, synthetic construct
  source 1..20: mol_type = other DNA
cgagtgcctgtttcatccag

SEQ ID NO: 55 - DNA, 52 bp, synthetic construct
  source 1..52: mol_type = other DNA
ttccagtgggcgctattctgctgttaggagacgaagtgataggacagggatg

SEQ ID NO: 56 - DNA, 20 bp, synthetic construct
  source 1..20: mol_type = other DNA
cagaatagcgcccactggaa

SEQ ID NO: 57 - DNA, 52 bp, synthetic construct
  source 1..52: mol_type = other DNA
ttccagtgggcgctattctgcctgcgccaccagaagtgataggacagggatg

SEQ ID NO: 58 - DNA, 20 bp, synthetic construct
  source 1..20: mol_type = other DNA
cagaatagcgcccactggaa

SEQ ID NO: 59 - DNA, 50 bp, synthetic construct
  source 1..50: mol_type = other DNA
ccagtgggcgctattctggtccgcgggacggaagtgataggacagggatg

SEQ ID NO: 60 - DNA, 20 bp, synthetic construct
  source 1..20: mol_type = other DNA
cagaatagcgcccactggaa

SEQ ID NO: 61 - protein, 1367 aa, synthetic construct
DKKYSIGLAIGTNSVGWAVITDEYKVPSKKFKVLGNTDRHSIKKNLIGALLFDSGETAEATRLKRTARRRYTRRKNRICYLQEIFSNEMAKVDDSFFHRLEESFLVEEDKKHERHPIFGNIVDEVAYHEKYPTIYHLRKKLVDSTDKADLRLIYLALAHMIKFRGHFLIEGDLNPDNSDVDKLFIQLVQTYNQLFEENPINASGVDAKAILSARLSKSRRLENLIAQLPGEKKNGLFGNLIALSLGLTPNFKSNFDLAEDAKLQLSKDTYDDDLDNLLAQIGDQYADLFLAAKNLSDAILLSDILRVNTEITKAPLSASMIKRYDEHHQDLTLLKALVRQQLPEKYKEIFFDQSKNGYAGYIDGGASQEEFYKFIKPILEKMDGTEELLVKLNREDLLRKQRTFDNGSIPHQIHLGELHAILRRQEDFYPFLKDNREKIEKILTFRIPYYVGPLARGNSRFAWMTRKSEETITPWNFEEVVDKGASAQSFIERMTNFDKNLPNEKVLPKHSLLYEYFTVYNELTKVKYVTEGMRKPAFLSGEQKKAIVDLLFKTNRKVTVKQLKEDYFKKIECFDSVEISGVEDRFNASLGTYHDLLKIIKDKDFLDNEENEDILEDIVLTLTLFEDREMIEERLKTYAHLFDDKVMKQLKRRRYTGWGRLSRKLINGIRDKQSGKTILDFLKSDGFANRNFMQLIHDDSLTFKEDIQKAQVSGQGDSLHEHIANLAGSPAIKKGILQTVKVVDELVKVMGRHKPENIVIEMARENQTTQKGQKNSRERMKRIEEGIKELGSQILKEHPVENTQLQNEKLYLYYLQNGRDMYVDQELDINRLSDYDVDHIVPQSFLKDDSIDNKVLTRSDKNRGKSDNVPSEEVVKKMKNYWRQLLNAKLITQRKFDNLTKAERGGLSELDKAGFIKRQLVETRQITKHVAQILDSRMNTKYDENDKLIREVKVITLKSKLVSDFRKDFQFYKVREINNYHHAHDAYLNAVVGTALIKKYPKLESEFVYGDYKVYDVRKMIAKSEQEIGKATAKYFFYSNIMNFFKTEITLANGEIRKRPLIETNGETGEIVWDKGRDFATVRKVLSMPQVNIVKKTEVQTGGFSKESILPKRNSDKLIARKKDWDPKKYGGFDSPTVAYSVLVVAKVEKGKSKKLKSVKELLGITIMERSSFEKNPIDFLEAKGYKEVKKDLIIKLPKYSLFELENGRKRMLASAGELQKGNELALPSKYVNFLYLASHYEKLKGSPEDNEQKQLFVEQHKHYLDEIIEQISEFSKRVILADANLDKVLSAYNKHRDKPIREQAENIIHLFTLTNLGAPAAFKYFDTTIDRKRYTSTKEVLDATLIHQSITGLYETRIDLSQLGGD

SEQ ID NO: 62 - DNA, 4101 bp, synthetic construct
  source 1..4101: mol_type = other DNA
gacaagaagtacagcatcggcctggccatcggcaccaactctgtgggctgggccgtgatcaccgacgagtacaaggtgcccagcaagaaattcaaggtgctgggcaacaccgaccggcacagcatcaagaagaacctgatcggagccctgctgttcgacagcggcgaaacagccgaggccacccggctgaagagaaccgccagaagaagatacaccagacggaagaaccggatctgctatctgcaagagatcttcagcaacgagatggccaaggtggacgacagcttcttccacagactggaagagtccttcctggtggaagaggataagaagcacgagcggcaccccatcttcggcaacatcgtggacgaggtggcctaccacgagaagtaccccaccatctaccacctgagaaagaaactggtggacagcaccgacaaggccgacctgcggctgatctatctggccctggcccacatgatcaagttccggggccacttcctgatcgagggcgacctgaaccccgacaacagcgacgtggacaagctgttcatccagctggtgcagacctacaaccagctgttcgaggaaaaccccatcaacgccagcggcgtggacgccaaggccatcctgtctgccagactgagcaagagcagacggctggaaaatctgatcgcccagctgcccggcgagaagaagaatggcctgttcggaaacctgattgccctgagcctgggcctgacccccaacttcaagagcaacttcgacctggccgaggatgccaaactgcagctgagcaaggacacctacgacgacgacctggacaacctgctggcccagatcggcgaccagtacgccgacctgtttctggccgccaagaacctgtccgacgccatcctgctgagcgacatcctgagagtgaacaccgagatcaccaaggcccccctgagcgcctctatgatcaagagatacgacgagcaccaccaggacctgaccctgctgaaagctctcgtgcggcagcagctgcctgagaagtacaaagagattttcttcgaccagagcaagaacggctacgccggctacattgacggcggagccagccaggaagagttctacaagttcatcaagcccatcctggaaaagatggacggcaccgaggaactgctcgtgaagctgaacagagaggacctgctgcggaagcagcggaccttcgacaacggcagcatcccccaccagatccacctgggagagctgcacgccattctgcggcggcaggaagatttttacccattcctgaaggacaaccgggaaaagatcgagaagatcctgaccttccgcatcccctactacgtgggccctctggccaggggaaacagcagattcgcctggatgaccagaaagagcgaggaaaccatcaccccctggaacttcgaggaagtggtggacaagggcgcttccgcccagagcttcatcgagcggatgaccaacttcgataagaacctgcccaacgagaaggtgctgcccaagcacagcctgctgtacgagtacttcaccgtgtataacgagctgaccaaagtgaaatacgtgaccgagggaatgagaaagcccgccttcctgagcggcgagcagaaaaaggccatcgtggacctgctgttcaagaccaaccggaaagtgaccgtgaagcagctgaaagaggactacttcaagaaaatcgagtgcttcgactccgtggaaatctccggcgtggaagatcggttcaacgcctccctgggcacataccacgatctgctgaaaattatcaaggacaaggacttcctggacaatgaggaaaacgaggacattctggaagatatcgtgctgaccctgacactgtttgaggacagagagatgatcgaggaacggctgaaaacctatgcccacctgttcgacgacaaagtgatgaagcagctgaagcggcggagatacaccggctggggcaggctgagccggaagctgatcaacggcatccgggacaagcagtccggcaagacaatcctggatttcctgaagtccgacggcttcgccaacagaaacttcatgcagctgatccacgacgacagcctgacctttaaagaggacatccagaaagcccaggtgtccggccagggcgatagcctgcacgagcacattgccaatctggccggcagccccgccattaagaagggcatcctgcagacagtgaaggtggtggacgagctcgtgaaagtgatgggccggcacaagcccgagaacatcgtgatcgaaatggccagagagaaccagaccacccagaagggacagaagaacagccgcgagagaatgaagcggatcgaagagggcatcaaagagctgggcagccagatcctgaaagaacaccccgtggaaaacacccagctgcagaacgagaagctgtacctgtactacctgcagaatgggcgggatatgtacgtggaccaggaactggacatcaaccggctgtccgactacgatgtggaccatatcgtgcctcagagctttctgaaggacgactccatcgacaacaaggtgctgaccagaagcgacaagaaccggggcaagagcgacaacgtgccctccgaagaggtcgtgaagaagatgaagaactactggcggcagctgctgaacgccaagctgattacccagagaaagttcgacaatctgaccaaggccgagagaggcggcctgagcgaactggataaggccggcttcatcaagagacagctggtggaaacccggcagatcacaaagcacgtggcacagatcctggactcccggatgaacactaagtacgacgagaatgacaagctgatccgggaagtgaaagtgatcaccctgaagtccaagctggtgtccgatttccggaaggatttccagttttacaaagtgcgcgagatcaacaactaccaccacgcccacgacgcctacctgaacgccgtcgtgggaaccgccctgatcaaaaagtaccctaagctggaaagcgagttcgtgtacggcgactacaaggtgtacgacgtgcggaagatgatcgccaagagcgagcaggaaatcggcaaggctaccgccaagtacttcttctacagcaacatcatgaactttttcaagaccgagattaccctggccaacggcgagatccggaagcggcctctgatcgagacaaacggcgaaaccggggagatcgtgtgggataagggccgggattttgccaccgtgcggaaagtgctgagcatgccccaagtgaatatcgtgaaaaagaccgaggtgcagacaggcggcttcagcaaagagtctatcctgcccaagaggaacagcgataagctgatcgccagaaagaaggactgggaccctaagaagtacggcggcttcgacagccccaccgtggcctattctgtgctggtggtggccaaagtggaaaagggcaagtccaagaaactgaagagtgtgaaagagctgctggggatcaccatcatggaaagaagcagcttcgagaagaatcccatcgactttctggaagccaagggctacaaagaagtgaaaaaggacctgatcatcaagctgcctaagtactccctgttcgagctggaaaacggccggaagagaatgctggcctctgccggcgaactgcagaagggaaacgaactggccctgccctccaaatatgtgaacttcctgtacctggccagccactatgagaagctgaagggctcccccgaggataatgagcagaaacagctgtttgtggaacagcacaagcactacctggacgagatcatcgagcagatcagcgagttctccaagagagtgatcctggccgacgctaatctggacaaagtgctgtccgcctacaacaagcaccgggataagcccatcagagagcaggccgagaatatcatccacctgtttaccctgaccaatctgggagcccctgccgccttcaagtactttgacaccaccatcgaccggaagaggtacaccagcaccaaagaggtgctggacgccaccctgatccaccagagcatcaccggcctgtacgagacacggatcgacctgtctcagctgggaggtgac

SEQ ID NO: 63 - DNA, 52 bp, synthetic construct
  source 1..52: mol_type = other DNA
ttccagtgggcgctattctgataatagatcaagaagtgataggacagggatg

SEQ ID NO: 64 - DNA, 20 bp, synthetic construct
  source 1..20: mol_type = other DNA
cagaatagcgcccactggaa

SEQ ID NO: 65 - DNA, 48 bp, synthetic construct
  source 1..48: mol_type = other DNA
ccagtgggcgctattctggttatggaaaatgaagtgataggacaggga

SEQ ID NO: 66 - DNA, 20 bp, synthetic construct
  source 1..20: mol_type = other DNA
cagaatagcgcccactggaa

SEQ ID NO: 67 - DNA, 52 bp, synthetic construct
  source 1..52: mol_type = other DNA
ttccagtgggcgctattctgattctaagaggggaagtgataggacagggatg

SEQ ID NO: 68 - DNA, 20 bp, synthetic construct
  source 1..20: mol_type = other DNA
cagaatagcgcccactggaa

SEQ ID NO: 69 - DNA, 52 bp, synthetic construct
  source 1..52: mol_type = other DNA
taggacagggatggaatagatcgattggcaatcacgaccccaccgcccacgc

SEQ ID NO: 70 - DNA, 20 bp, synthetic construct
  source 1..20: mol_type = other DNA
tctattccatccctgtccta

SEQ ID NO: 71 - DNA, 52 bp, synthetic construct
  source 1..52: mol_type = other DNA
taggacagggatggaatagaaataaccaatcacacgaccccaccgcccacgc

SEQ ID NO: 72 - DNA, 20 bp, synthetic construct
  source 1..20: mol_type = other DNA
tctattccatccctgtccta

SEQ ID NO: 73 - DNA, 50 bp, synthetic construct
  source 1..50: mol_type = other DNA
ggacagggatggaatagagctgtacgaaaacacgaccccaccgcccacgc

SEQ ID NO: 74 - DNA, 20 bp, synthetic construct
  source 1..20: mol_type = other DNA
tctattccatccctgtccta

SEQ ID NO: 75 - DNA, 52 bp, synthetic construct
  source 1..52: mol_type = other DNA
taggacagggatggaatagatgttacgcccatcacgaccccaccgcccacgc

SEQ ID NO: 76 - DNA, 20 bp, synthetic construct
  source 1..20: mol_type = other DNA
tctattccatccctgtccta

SEQ ID NO: 77 - DNA, 52 bp, synthetic construct
  source 1..52: mol_type = other DNA
taggacagggatggaatagatcgggctatgcccacgaccccaccgcccacgc

SEQ ID NO: 78 - DNA, 20 bp, synthetic construct
  source 1..20: mol_type = other DNA
tctattccatccctgtccta

SEQ ID NO: 79 - DNA, 52 bp, synthetic construct
  source 1..52: mol_type = other DNA
taggacagggatggaatagaaaccgcgtttcacacgaccccaccgcccacgc

SEQ ID NO: 80 - DNA, 20 bp, synthetic construct
  source 1..20: mol_type = other DNA
tctattccatccctgtccta

SEQ ID NO: 81 - DNA, 37 bp, synthetic construct
  source 1..37: mol_type = other DNA
acgccaccctgtacgtgatcttcgagccctgcgtgat

SEQ ID NO: 82 - DNA, 18 bp, synthetic construct
  source 1..18: mol_type = other DNA
tcacgtacagggtggcgt

SEQ ID NO: 83 - DNA, 37 bp, synthetic construct
  source 1..37: mol_type = other DNA
tgtacgtgaccttcgagctctgcgtgatgtgcgccgg

SEQ ID NO: 84 - DNA, 18 bp, synthetic construct
  source 1..18: mol_type = other DNA
gctcgaaggtcacgtaca

SEQ ID NO: 85 - DNA, 37 bp, synthetic construct
  source 1..37: mol_type = other DNA
ctgtacgtgaccttcgagtcctgcgtgatgtgcgccg

SEQ ID NO: 86 - DNA, 18 bp, synthetic construct
  source 1..18: mol_type = other DNA
ctcgaaggtcacgtacag

SEQ ID NO: 87 - DNA, 57 bp, synthetic construct
  source 1..57: mol_type = other DNA
ggctacggtctcaagcgagatgctgtgggcgtgcatacagcagcctagggaagtgtt

SEQ ID NO: 88 - DNA, 44 bp, synthetic construct
  source 1..44: mol_type = other DNA
ggctacggtctcacgctgcactcgttggccatcacgccggcggt

SEQ ID NO: 89 - DNA, 57 bp, synthetic construct
  source 1..57: mol_type = other DNA
ggctacggtctcaagcgagatgctggcgcaattttggcagcagcctagggaagtgtt

SEQ ID NO: 90 - DNA, 44 bp, synthetic construct; identical to SEQ ID NO: 88
  source 1..44: mol_type = other DNA

SEQ ID NO: 91 - DNA, 57 bp, synthetic construct
  source 1..57: mol_type = other DNA
ggctacggtctcaagcgagatgctgttctggtactatcagcagcctagggaagtgtt

SEQ ID NO: 92 - DNA, 44 bp, synthetic construct; identical to SEQ ID NO: 88
  source 1..44: mol_type = other DNA

SEQ ID NO: 93 - DNA, 57 bp, synthetic construct
  source 1..57: mol_type = other DNA
ggctacggtctcaagcgagatgctgagtaggcgcggtcagcagcctagggaagtgtt

SEQ ID NO: 94 - DNA, 44 bp, synthetic construct; identical to SEQ ID NO: 88
  source 1..44: mol_type = other DNA

SEQ ID NO: 95 - DNA, 37 bp, synthetic construct
  source 1..37: mol_type = other DNA
ccctgtacgtgaccttcgcgccctgcgtgatgtgcgc

SEQ ID NO: 96 - DNA, 18 bp, synthetic construct
  source 1..18: mol_type = other DNA
cgaaggtcacgtacaggg

SEQ ID NO: 97 - DNA, 37 bp, synthetic construct
  source 1..37: mol_type = other DNA
acgccaccctgtacgtgaacttcgagccctgcgtgat

SEQ ID NO: 98 - DNA, 18 bp, synthetic construct
  source 1..18: mol_type = other DNA
tcacgtacagggtggcgt

SEQ ID NO: 99 - DNA, 37 bp, synthetic construct
  source 1..37: mol_type = other DNA
accctgtacgtgaccttccagccctgcgtgatgtgcg

SEQ ID NO: 100 - DNA, 18 bp, synthetic construct
  source 1..18: mol_type = other DNA
tcacgtacagggtggcgt

SEQ ID NO: 101 - DNA, 37 bp, synthetic construct
  source 1..37: mol_type = other DNA
gagactggtctacggcgtaagcaactcaaaaagaggc

SEQ ID NO: 102 - DNA, 18 bp, synthetic construct
  source 1..18: mol_type = other DNA
acgccgtagaccagtctc

SEQ ID NO: 103 - DNA, 37 bp, synthetic construct
  source 1..37: mol_type = other DNA
agagactggtctacggcgcgagcaactcaaaaagagg

SEQ ID NO: 104 - DNA, 18 bp, synthetic construct
  source 1..18: mol_type = other DNA
agagactggtctacggcg

SEQ ID NO: 105 - DNA, 37 bp, synthetic construct
  source 1..37: mol_type = other DNA
gactggtctacggcgtgatcaactcaaaaagaggcgc

SEQ ID NO: 106 - DNA, 18 bp, synthetic construct
  source 1..18: mol_type = other DNA
tcacgccgtagaccagtc

SEQ ID NO: 107 - DNA, 37 bp, synthetic construct
  source 1..37: mol_type = other DNA
ctggtctacggcgtgagccactcaaaaagaggcgccg

SEQ ID NO: 108 - DNA, 18 bp, synthetic construct
  source 1..18: mol_type = other DNA
gctcacgccgtagaccag

SEQ ID NO: 109 - DNA, 37 bp, synthetic construct
  source 1..37: mol_type = other DNA
agactggtctacggcgtgcgcaactcaaaaagaggcg

SEQ ID NO: 110 - DNA, 18 bp, synthetic construct
  source 1..18: mol_type = other DNA
cacgccgtagaccagtct

SEQ ID NO: 111 - DNA, 48 bp, synthetic construct
  source 1..48: mol_type = other DNA
ctacggcgtgagcaactcaaggcggggagccgccggcagcctgctgaa

SEQ ID NO: 112 - DNA, 20 bp, synthetic construct
  source 1..20: mol_type = other DNA
ttgagttgctcacgccgtag

SEQ ID NO: 113 - DNA, 52 bp, synthetic construct
  source 1..52: mol_type = other DNA
tggtctacggcgtgagcaacactggccttgctgccgccggcagcctgctgaa

SEQ ID NO: 114 - DNA, 20 bp, synthetic construct
  source 1..20: mol_type = other DNA
gttgctcacgccgtagacca

SEQ ID NO: 115 - DNA, 51 bp, synthetic construct
  source 1..51: mol_type = other DNA
ggtctacggcgtgagcaactacgaaggaggagccgccggcagcctgctgaa

SEQ ID NO: 116 - DNA, 20 bp, synthetic construct
  source 1..20: mol_type = other DNA
ttgagttgctcacgccgtag

SEQ ID NO: 117 - DNA, 51 bp, synthetic construct; identical to SEQ ID NO: 115
  source 1..51: mol_type = other DNA

SEQ ID NO: 118 - DNA, 20 bp, synthetic construct
  source 1..20: mol_type = other DNA
ttgagttgctcacgccgtag

SEQ ID NO: 119 - DNA, 52 bp, synthetic construct
  source 1..52: mol_type = other DNA
tggtctacggcgtgagcaacagtctaaagcgggccgccggcagcctgctgaa

SEQ ID NO: 120 - DNA, 20 bp, synthetic construct
  source 1..20: mol_type = other DNA
ttgagttgctcacgccgtag

SEQ ID NO: 121 - DNA, 65 bp, synthetic construct
  source 1..65: mol_type = other DNA
ggctacggtctcagaggcgccgccggcagcctgctgaccgtgctgaactaccccggcatgaacca

SEQ ID NO: 122 - DNA, 49 bp, synthetic construct
  source 1..49: mol_type = other DNA
ggctacggtctcacctctttttgagttgctcacgccgtagaccagtctc

SEQ ID NO: 123 - DNA, 65 bp, synthetic construct
  source 1..65: mol_type = other DNA
ggctacggtctcagaggcgccgccggcagcctgctgaacgtgcggaactaccccggcatgaacca

SEQ ID NO: 124 - DNA, 49 bp, synthetic construct; identical to SEQ ID NO: 122
  source 1..49: mol_type = other DNA

SEQ ID NO: 125 - DNA, 65 bp, synthetic construct
  source 1..65: mol_type = other DNA
ggctacggtctcagaggcgccgccggcagcctgctgaacgggctgaactaccccggcatgaacca

SEQ ID NO: 126 - DNA, 49 bp, synthetic construct; identical to SEQ ID NO: 122
  source 1..49: mol_type = other DNA

SEQ ID NO: 127 - DNA, 57 bp, synthetic construct
  source 1..57: mol_type = other DNA
ggctacggtctcactgaacgtgctgaactcccccggcatgaaccaccagatcgagat

SEQ ID NO: 128 - DNA, 49 bp, synthetic construct
  source 1..49: mol_type = other DNA
ggctacggtctcatcagcaggctgccggcggcgcctctttttgagttgc

SEQ ID NO: 129 - DNA, 57 bp, synthetic construct
  source 1..57: mol_type = other DNA
ggctacggtctcactgaacgtgctgggcagtaaatccatgaaccaccagatcgagat

SEQ ID NO: 130 - DNA, 49 bp, synthetic construct; identical to SEQ ID NO: 128
  source 1..49: mol_type = other DNA

SEQ ID NO: 131 - DNA, 57 bp, synthetic construct
  source 1..57: mol_type = other DNA
ggctacggtctcactgaacgtgctggactaccccggcatgaaccaccagatcgagat

SEQ ID NO: 132 - DNA, 49 bp, synthetic construct; identical to SEQ ID NO: 128
  source 1..49: mol_type = other DNA

SEQ ID NO: 133 - DNA, 57 bp, synthetic construct
  source 1..57: mol_type = other DNA
ggctacggtctcactgaacgtgctgaaatatgctacgatgaaccaccagatcgagat

SEQ ID NO: 134 - DNA, 49 bp, synthetic construct; identical to SEQ ID NO: 128
  source 1..49: mol_type = other DNA

SEQ ID NO: 135 - DNA, 57 bp, synthetic construct
  source 1..57: mol_type = other DNA
ggctacggtctcactgaacgtgctgggccttccgttaatgaaccaccagatcgagat

SEQ ID NO: 136 - DNA, 49 bp, synthetic construct; identical to SEQ ID NO: 128
  source 1..49: mol_type = other DNA

SEQ ID NO: 137 - DNA, 57 bp, synthetic construct
  source 1..57: mol_type = other DNA
ggctacggtctcaagcgagatgctgttttcagtcttacagcagcctagggaagtgtt

SEQ ID NO: 138 - DNA, 44 bp, synthetic construct; identical to SEQ ID NO: 88
  source 1..44: mol_type = other DNA

SEQ ID NO: 139 - DNA, 57 bp, synthetic construct
  source 1..57: mol_type = other DNA
ggctacggtctcatgccagttctatgggggggtgaaggaagtgttcaatgctgagcg

SEQ ID NO: 140 - DNA, 33 bp, synthetic construct; identical to SEQ ID NO: 6
  source 1..33: mol_type = other DNA

SEQ ID NO: 141 - RNA, 33 nt, synthetic construct
  source 1..33: mol_type = other RNA
ggctacggtctcaggcacagcatctcgctgcac

SEQ ID NO: 142 - RNA, 20 nt, synthetic construct
  source 1..20: mol_type = other RNA
gaacacaaagcatagactgc

SEQ ID NO: 143 - RNA, 19 nt, synthetic construct
  source 1..19: mol_type = other RNA
taaacaaagcatagactga

SEQ ID NO: 144 - RNA, 19 nt, synthetic construct
  source 1..19: mol_type = other RNA
ggaataaatcatagaatcc

SEQ ID NO: 145 - RNA, 20 nt, synthetic construct
  source 1..20: mol_type = other RNA
acacacacacttagaatctg

SEQ ID NO: 146 - DNA, 17 bp, synthetic construct
  source 1..17: mol_type = other DNA
gctagccttgcgttccg

SEQ ID NO: 147 - DNA, 19 bp, synthetic construct
  source 1..19: mol_type = other DNA
gtccccaagatcgtgccaa

SEQ ID NO: 148 - DNA, 20 bp, synthetic construct
  source 1..20: mol_type = other DNA
cctcagcattcagccactaa

SEQ ID NO: 149 - DNA, 20 bp, synthetic construct
  source 1..20: mol_type = other DNA
agaggcccattaacgtttgg

SEQ ID NO: 150 - DNA, 20 bp, synthetic construct
  source 1..20: mol_type = other DNA
ttccttctacggcagaaacc

SEQ ID NO: 151 - DNA, 20 bp, synthetic construct
  source 1..20: mol_type = other DNA
aacaagtagcaacaggaggg

SEQ ID NO: 152 - DNA, 20 bp, synthetic construct
  source 1..20: mol_type = other DNA
gggaacaaaccaggcataca

SEQ ID NO: 153 - DNA, 20 bp, synthetic construct
  source 1..20: mol_type = other DNA
cctcaaggaacaacctgtcc

SEQ ID NO: 154 - DNA, 20 bp, synthetic construct
  source 1..20: mol_type = other DNA
gagaggctgccaagctaaat

SEQ ID NO: 155 - DNA, 20 bp, synthetic construct
  source 1..20: mol_type = other DNA
tggagctcaagatcacgttg

SEQ ID NO: 156 - protein, 540 aa, synthetic construct
ATGTACAATGCCCCTAGATTCTTTTGTAGATCTGCTGCCGTGTCTGATCATGAGTTTAACGATGAGTACTGGATGAGACACGCCCTGACACTGGCCAAGAGGGCTCGGGAGGAAGGAGAGGTGCCAGTGGGAGCTGTGCTGGTGCTGAATAATCAGGTCATTGGAGAAGGATGGAATAGAGCCATCGGCCTGCACGACCCCACCGCCCACGCCGAGATCATGGCCCTGAGACAGGGCGGCCTGGTGCTGCAGAACTACCGGCTGATCGACGCCACCCTGTACGTGACCTTCGAGCCCTGCGTGATGTGCGCCGGCGCCATGGTGCATAGCAGAATCAGCAGACTGGTGTTCGGCGTGAGAAACTCAAAGAGAGGCGCCGCCGGCAGCCTGATCAACGTGCTGAACTACCCCGGCATGAACCACAGAGTGGAGATCACCGAGGGCATCCTGGCCGAGAGCTGCAGCGCCATGCTGTGCGACTTCTATAGGTGGCCTAGGGAGGTGTTCAATGCCCTGAAGAAGGCCAGACAGGAGGAGGGC

SEQ ID NO: 157 - DNA, 4857 bp, synthetic construct
  source 1..4857: mol_type = other DNA
atgaaacggacagccgacggaagcgagttcgagtcaccaaagaagaagcggaaagtcatgtacaatgcccctagattcttttgtagatctgctgccgtgtctgatcatgagtttaacgatgagtactggatgagacacgccctgacactggccaagagggctcgggaggaaggagaggtgccagtgggagctgtgctggtgctgaataatcaggtcattggagaaggatggaatagagccatcggcctgcacgaccccaccgcccacgccgagatcatggccctgagacagggcggcctggtgctgcagaactaccggctgatcgacgccaccctgtacgtgaccttcgagccctgcgtgatgtgcgccggcgccatggtgcatagcagaatcagcagactggtgttcggcgtgagaaactcaaagagaggcgccgccggcagcctgatcaacgtgctgaactaccccggcatgaaccacagagtggagatcaccgagggcatcctggccgagagctgcagcgccatgctgtgcgacttctataggtggcctagggaggtgttcaatgccctgaagaaggccagacaggaggagggctccggaggatctagcggaggctcctctggctctgagacacctggcacaagcgagagcgcaacacctgaaagcagcgggggcagcagcggggggtcagacaagaagtacagcatcggcctggccatcggcaccaactctgtgggctgggccgtgatcaccgacgagtacaaggtgcccagcaagaaattcaaggtgctgggcaacaccgaccggcacagcatcaagaagaacctgatcggagccctgctgttcgacagcggcgaaacagccgaggccacccggctgaagagaaccgccagaagaagatacaccagacggaagaaccggatctgctatctgcaagagatcttcagcaacgagatggccaaggtggacgacagcttcttccacagactggaagagtccttcctggtggaagaggataagaagcacgagcggcaccccatcttcggcaacatcgtggacgaggtggcctaccacgagaagtaccccaccatctaccacctgagaaagaaactggtggacagcaccgacaaggccgacctgcggctgatctatctggccctggcccacatgatcaagttccggggccacttcctgatcgagggcgacctgaaccccgacaacagcgacgtggacaagctgttcatccagctggtgcagacctacaaccagctgttcgaggaaaaccccatcaacgccagcggcgtggacgccaaggccatcctgtctgccagactgagcaagagcagacggctggaaaatctgatcgcccagctgcccggcgagaagaagaatggcctgttcggaaacctgattgccctgagcctgggcctgacccccaacttcaagagcaacttcgacctggccgaggatgccaaactgcagctgagcaaggacacctacgacgacgacctggacaacctgctggcccagatcggcgaccagtacgccgacctgtttctggccgccaagaacctgtccgacgccatcctgctgagcgacatcctgagagtgaacaccgagatcaccaaggcccccctgagcgcctctatgatcaagagatacgacgagcaccaccaggacctgaccctgctgaaagctctcgtgcggcagcagctgcctgagaagtacaaagagattttcttcgaccagagcaagaacggctacgccggctacattgacggcggagccagccaggaagagttctacaagttcatcaagcccatcctggaaaagatggacggcaccgaggaactgctcgtgaagctgaacagagaggacctgctgcggaagcagcggaccttcgacaacggcagcatcccccaccagatccacctgggagagctgcacgccattctgcggcggcaggaagatttttacccattcctgaaggacaaccgggaaaagatcgagaagatcctgaccttccgcatcccctactacgtgggccctctggccaggggaaacagcagattcgcctggatgaccagaaagagcgaggaaaccatcaccccctggaacttcgaggaagtggtggacaagggcgcttccgcccagagcttcatcgagcggatgaccaacttcgataagaacctgcccaacgagaaggtgctgcccaagcacagcctgctgtacgagtacttcaccgtgtataacgagctgaccaaagtgaaatacgtgaccgagggaatgagaaagcccgccttcctgagcggcgagcagaaaaaggccatcgtggacctgctgttcaagaccaaccggaaagtgaccgtgaagcagctgaaagaggactacttcaagaaaatcgagtgcttcgactccgtggaaatctccggcgtggaagatcggttcaacgcctccctgggcacataccacgatctgctgaaaattatcaaggacaaggacttcctggacaatgaggaaaacgaggacattctggaagatatcgtgctgaccctgacactgtttgaggacagagagatgatcgaggaacggctgaaaacctatgcccacctgttcgacgacaaagtgatgaagcagctgaagcggcggagatacaccggctggggcaggctgagccggaagctgatcaacggcatccgggacaagcagtccggcaagacaatcctggatttcctgaagtccgacggcttcgccaacagaaacttcatgcagctgatccacgacgacagcctgacctttaaagaggacatccagaaagcccaggtgtccggccagggcgatagcctgcacgagcacattgccaatctggccggcagccccgccattaagaagggcatcctgcagacagtgaaggtggtggacgagctcgtgaaagtgatgggccggcacaagcccgagaacatcgtgatcgaaatggccagagagaaccagaccacccagaagggacagaagaacagccgcgagagaatgaagcggatcgaagagggcatcaaagagctgggcagccagatcctgaaagaacaccccgtggaaaacacccagctgcagaacgagaagctgtacctgtactacctgcagaatgggcgggatatgtacgtggaccaggaactggacatcaaccggctgtccgactacgatgtggaccatatcgtgcctcagagctttctgaaggacgactccatcgacaacaaggtgctgaccagaagcgacaagaaccggggcaagagcgacaacgtgccctccgaagaggtcgtgaagaagatgaagaactactggcggcagctgctgaacgccaagctgattacccagagaaagttcgacaatctgaccaaggccgagagaggcggcctgagcgaactggataaggccggcttcatcaagagacagctggtggaaacccggcagatcacaaagcacgtggcacagatcctggactcccggatgaacactaagtacgacgagaatgacaagctgatccgggaagtgaaagtgatcaccctgaagtccaagctggtgtccgatttccggaaggatttccagttttacaaagtgcgcgagatcaacaactaccaccacgcccacgacgcctacctgaacgccgtcgtgggaaccgccctgatcaaaaagtaccctaagctggaaagcgagttcgtgtacggcgactacaaggtgtacgacgtgcggaagatgatcgccaagagcgagcaggaaatcggcaaggctaccgccaagtacttcttctacagcaacatcatgaactttttcaagaccgagattaccctggccaacggcgagatccggaagcggcctctgatcgagacaaacggcgaaaccggggagatcgtgtgggataagggccgggattttgccaccgtgcggaaagtgctgagcatgccccaagtgaatatcgtgaaaaagaccgaggtgcagacaggcggcttcagcaaagagtctatcctgcccaagaggaacagcgataagctgatcgccagaaagaaggactgggaccctaagaagtacggcggcttcgacagccccaccgtggcctattctgtgctggtggtggccaaagtggaaaagggcaagtccaagaaactgaagagtgtgaaagagctgctggggatcaccatcatggaaagaagcagcttcgagaagaatcccatcgactttctggaagccaagggctacaaagaagtgaaaaaggacctgatcatcaagctgcctaagtactccctgttcgagctggaaaacggccggaagagaatgctggcctctgccggcgaactgcagaagggaaacgaactggccctgccctccaaatatgtgaacttcctgtacctggccagccactatgagaagctgaagggctcccccgaggataatgagcagaaacagctgtttgtggaacagcacaagcactacctggacgagatcatcgagcagatcagcgagttctccaagagagtgatcctggccgacgctaatctggacaaagtgctgtccgcctacaacaagcaccgggataagcccatcagagagcaggccgagaatatcatccacctgtttaccctgaccaatctgggagcccctgccgccttcaagtactttgacaccaccatcgaccggaagaggtacaccagcaccaaagaggtgctggacgccaccctgatccaccagagcatcaccggcctgtacgagacacggatcgacctgtctcagctgggaggtgactctggcggctcaaaaagaaccgccgacggcagcgaattcgagcccaagaagaagaggaaagtc

SEQ ID NO: 158 - DNA, 4857 bp, synthetic construct
  source 1..4857: mol_type = other DNA
atgaaacggacagccgacggaagcgagttcgagtcaccaaagaagaagcggaaagtcatgtacaatgcccctagattcttttgtagatctgctgccgtgacagagaaggaatatcaggatgagtactggatgagacacgccctgacactggccaagagggctcgggaggaaggagaggtgccagtgggagctgtgctggtgctgaataatcaggtcattggagaaggatggaatagagccatcggcctgcacgaccccaccgcccacgccgagatcatggccctgagacagggcggcctggtgctgcagaactaccggctgatcgacgccaccctgtacgtgaccttcgagccctgcgtgatgtgcgccggcgccatggtgcatagcagaatcagcagactggtgttcggcgtgagaaactcaaagagaggcgccgccggcagcctgatcaacgtgctgaactaccccggcatgaaccacagagtggagatcaccgagggcatcctggccgagagctgcagcgccatgctgtgcgacttctataggtggcctagggaggtgttcaatgccctgaagaaggccagacaggaggagggctccggaggatctagcggaggctcctctggctctgagacacctggcacaagcgagagcgcaacacctgaaagcagcgggggcagcagcggggggtcagacaagaagtacagcatcggcctggccatcggcaccaactctgtgggctgggccgtgatcaccgacgagtacaaggtgcccagcaagaaattcaaggtgctgggcaacaccgaccggcacagcatcaagaagaacctgatcggagccctgctgttcgacagcggcgaaacagccgaggccacccggctgaagagaaccgccagaagaagatacaccagacggaagaaccggatctgctatctgcaagagatcttcagcaacgagatggccaaggtggacgacagcttcttccacagactggaagagtccttcctggtggaagaggataagaagcacgagcggcaccccatcttcggcaacatcgtggacgaggtggcctaccacgagaagtaccccaccatctaccacctgagaaagaaactggtggacagcaccgacaaggccgacctgcggctgatctatctggccctggcccacatgatcaagttccggggccacttcctgatcgagggcgacctgaaccccgacaacagcgacgtggacaagctgttcatccagctggtgcagacctacaaccagctgttcgaggaaaaccccatcaacgccagcggcgtggacgccaaggccatcctgtctgccagactgagcaagagcagacggctggaaaatctgatcgcccagctgcccggcgagaagaagaatggcctgttcggaaacctgattgccctgagcctgggcctgacccccaacttcaagagcaacttcgacctggccgaggatgccaaactgcagctgagcaaggacacctacgacgacgacctggacaacctgctggcccagatcggcgaccagtacgccgacctgtttctggccgccaagaacctgtccgacgccatcctgctgagcgacatcctgagagtgaacaccgagatcaccaaggcccccctgagcgcctctatgatcaagagatacgacgagcaccaccaggacctgaccctgctgaaagctctcgtgcggcagcagctgcctgagaagtacaaagagattttcttcgaccagagcaagaacggctacgccggctacattgacggcggagccagccaggaagagttctacaagttcatcaagcccatcctggaaaagatggacggcaccgaggaactgctcgtgaagctgaacagagaggacctgctgcggaagcagcggaccttcgacaacggcagcatcccccaccagatccacctgggagagctgcacgccattctgcggcggcaggaagatttttacccattcctgaaggacaaccgggaaaagatcgagaagatcctgaccttccgcatcccctactacgtgggccctctggccaggggaaacagcagattcgcctggatgaccagaaagagcgaggaaaccatcaccccctggaacttcgaggaagtggtggacaagggcgcttccgcccagagcttcatcgagcggatgaccaacttcgataagaacctgcccaacgagaaggtgctgcccaagcacagcctgctgtacgagtacttcaccgtgtataacgagctgaccaaagtgaaatacgtgaccgagggaatgagaaagcccgccttcctgagcggcgagcagaaaaaggccatcgtggacctgctgttcaagaccaaccggaaagtgaccgtgaagcagctgaaagaggactacttcaagaaaatcgagtgcttcgactccgtggaaatctccggcgtggaagatcggttcaacgcctccctgggcacataccacgatctgctgaaaattatcaaggacaaggacttcctggacaatgaggaaaacgaggacattctggaagatatcgtgctgaccctgacactgtttgaggacagagagatgatcgaggaacggctgaaaacctatgcccacctgttcgacgacaaagtgatgaagcagctgaagcggcggagatacaccggctggggcaggctgagccggaagctgatcaacggcatccgggacaagcagtccggcaagacaatcctggatttcctgaagtccgacggcttcgccaacagaaacttcatgcagctgatccacgacgacagcctgacctttaaagaggacatccagaaagcccaggtgtccggccagggcgatagcctgcacgagcacattgccaatctggccggcagccccgccattaagaagggcatcctgcagacagtgaaggtggtggacgagctcgtgaaagtgatgggccggcacaagcccgagaacatcgtgatcgaaatggccagagagaaccagaccacccagaagggacagaagaacagccgcgagagaatgaagcggatcgaagagggcatcaaagagctgggcagccagatcctgaaagaacaccccgtggaaaacacccagctgcagaacgagaagctgtacctgtactacctgcagaatgggcgggatatgtacgtggaccaggaactggacatcaaccggctgtccgactacgatgtggaccatatcgtgcctcagagctttctgaaggacgactccatcgacaacaaggtgctgaccagaagcgacaagaaccggggcaagagcgacaacgtgccctccgaagaggtcgtgaagaagatgaagaactactggcggcagctgctgaacgccaagctgattacccagagaaagttcgacaatctgaccaaggccgagagaggcggcctgagcgaactggataaggccggcttcatcaagagacagctggtggaaacccggcagatcacaaagcacgtggcacagatcctggactcccggatgaacactaagtacgacgagaatgacaagctgatccgggaagtgaaagtgatcaccctgaagtccaagctggtgtccgatttccggaaggatttccagttttacaaagtgcgcgagatcaacaactaccaccacgcccacgacgcctacctgaacgccgtcgtgggaaccgccctgatcaaaaagtaccctaagctggaaagcgagttcgtgtacggcgactacaaggtgtacgacgtgcggaagatgatcgccaagagcgagcaggaaatcggcaaggctaccgccaagtacttcttctacagcaacatcatgaactttttcaagaccgagattaccctggccaacggcgagatccggaagcggcctctgatcgagacaaacggcgaaaccggggagatcgtgtgggataagggccgggattttgccaccgtgcggaaagtgctgagcatgccccaagtgaatatcgtgaaaaagaccgaggtgcagacaggcggcttcagcaaagagtctatcctgcccaagaggaacagcgataagctgatcgccagaaagaaggactgggaccctaagaagtacggcggcttcgacagccccaccgtggcctattctgtgctggtggtggccaaagtggaaaagggcaagtccaagaaactgaagagtgtgaaagagctgctggggatcaccatcatggaaagaagcagcttcgagaagaatcccatcgactttctggaagccaagggctacaaagaagtgaaaaaggacctgatcatcaagctgcctaagtactccctgttcgagctggaaaacggccggaagagaatgctggcctctgccggcgaactgcagaagggaaacgaactggccctgccctccaaatatgtgaacttcctgtacctggccagccactatgagaagctgaagggctcccccgaggataatgagcagaaacagctgtttgtggaacagcacaagcactacctggacgagatcatcgagcagatcagcgagttctccaagagagtgatcctggccgacgctaatctggacaaagtgctgtccgcctacaacaagcaccgggataagcccatcagagagcaggccgagaatatcatccacctgtttaccctgaccaatctgggagcccctgccgccttcaagtactttgacaccaccatcgaccggaagaggtacaccagcaccaaagaggtgctggacgccaccctgatccaccagagcatcaccggcctgtacgagacacggatcgacctgtctcagctgggaggtgactctggcggctcaaaaagaaccgccgacggcagcgaattcgagcccaagaagaagaggaaagtc

SEQ ID NO: 159 - DNA, 4857 bp, synthetic construct
  source 1..4857: mol_type = other DNA
atgaaacggacagccgacggaagcgagttcgagtcaccaaagaagaagcggaaagtcatgtacaatgcccctagattcttttgtagatctgctgccgtgtctgatcatgagtttaacgatgattttttcatgaagcgcgcaattacactggccaagagggctcgggaggaaggagaggtgccagtgggagctgtgctggtgctgaataatcaggtcattggagaaggatggaatagagccatcggcctgcacgaccccaccgcccacgccgagatcatggccctgagacagggcggcctggtgctgcagaactaccggctgatcgacgccaccctgtacgtgaccttcgagccctgcgtgatgtgcgccggcgccatggtgcatagcagaatcagcagactggtgttcggcgtgagaaactcaaagagaggcgccgccggcagcctgatcaacgtgctgaactaccccggcatgaaccacagagtggagatcaccgagggcatcctggccgagagctgcagcgccatgctgtgcgacttctataggtggcctagggaggtgttcaatgccctgaagaaggccagacaggaggagggctccggaggatctagcggaggctcctctggctctgagacacctggcacaagcgagagcgcaacacctgaaagcagcgggggcagcagcggggggtcagacaagaagtacagcatcggcctggccatcggcaccaactctgtgggctgggccgtgatcaccgacgagtacaaggtgcccagcaagaaattcaaggtgctgggcaacaccgaccggcacagcatcaagaagaacctgatcggagccctgctgttcgacagcggcgaaacagccgaggccacccggctgaagagaaccgccagaagaagatacaccagacggaagaaccggatctgctatctgcaagagatcttcagcaacgagatggccaaggtggacgacagcttcttccacagactggaagagtccttcctggtggaagaggataagaagcacgagcggcaccccatcttcggcaacatcgtggacgaggtggcctaccacgagaagtaccccaccatctaccacctgagaaagaaactggtggacagcaccgacaaggccgacctgcggctgatctatctggccctggcccacatgatcaagttccggggccacttcctgatcgagggcgacctgaaccccgacaacagcgacgtggacaagctgttcatccagctggtgcagacctacaaccagctgttcgaggaaaaccccatcaacgccagcggcgtggacgccaaggccatcctgtctgccagactgagcaagagcagacggctggaaaatctgatcgcccagctgcccggcgagaagaagaatggcctgttcggaaacctgattgccctgagcctgggcctgacccccaacttcaagagcaacttcgacctggccgaggatgccaaactgcagctgagcaaggacacctacgacgacgacctggacaacctgctggcccagatcggcgaccagtacgccgacctgtttctggccgccaagaacctgtccgacgccatcctgctgagcgacatcctgagagtgaacaccgagatcaccaaggcccccctgagcgcctctatgatcaagagatacgacgagcaccaccaggacctgaccctgctgaaagctctcgtgcggcagcagctgcctgagaagtacaaagagattttcttcgaccagagcaagaacggctacgccggctacattgacggcggagccagccaggaagagttctacaagttcatcaagcccatcctggaaaagatggacggcaccgaggaactgctcgtgaagctgaacagagaggacctgctgcggaagcagcggaccttcgacaacggcagcatcccccaccagatccacctgggagagctgcacgccattctgcggcggcaggaagatttttacccattcctgaaggacaaccgggaaaagatcgagaagatcctgaccttccgcatcccctactacgtgggccctctggccaggggaaacagcagattcgcctggatgaccagaaagagcgaggaaaccatcaccccctggaacttcgaggaagtggtggacaagggcgcttccgcccagagcttcatcgagcggatgaccaacttcgataagaacctgcccaacgagaaggtgctgcccaagcacagcctgctgtacgagtacttcaccgtgtataacgagctgaccaaagtgaaatacgtgaccgagggaatgagaaagcccgccttcctgagcggcgagcagaaaaaggccatcgtggacctgctgttcaagaccaaccggaaagtgaccgtgaagcagctgaaagaggactacttcaagaaaatcgagtgcttcgactccgtggaaatctccggcgtggaagatcggttcaacgcctccctgggcacataccacgatctgctgaaaattatcaaggacaaggacttcctggacaatgaggaaaacgaggacattctggaagatatcgtgctgaccctgacactgtttgaggacagagagatgatcgaggaacggctgaaaacctatgcccacctgttcgacgacaaagtgatgaagcagctgaagcggcggagatacaccggctggggcaggctgagccggaagctgatcaacggcatccgggacaagcagtccggcaagacaatcctggatttcctgaagtccgacggcttcgccaacagaaacttcatgcagctgatccacgacgacagcctgacctttaaagaggacatccagaaagcccaggtgtccggccagggcgatagcctgcacgagcacattgccaatctggccggcagccccgccattaagaagggcatcctgcagacagtgaaggtggtggacgagctcgtgaaagtgatgggccggcacaagcccgagaacatcgtgatcgaaatggccagagagaaccagaccacccagaagggacagaagaacagccgcgagagaatgaagcggatcgaagagggcatcaaagagctgggcagccagatcctgaaagaacaccccgtggaaaacacccagctgcagaacgagaagctgtacctgtactacctgcagaatgggcgggatatgtacgtggaccaggaactggacatcaaccggctgtccgactacgatgtggaccatatcgtgcctcagagctttctgaaggacgactccatcgacaacaaggtgctgaccagaagcgacaagaaccggggcaagagcgacaacgtgccctccgaagaggtcgtgaagaagatgaagaactactggcggcagctgctgaacgccaagctgattacccagagaaagttcgacaatctgaccaaggccgagagaggcggcctgagcgaactggataaggccggcttcatcaagagacagctggtggaaacccggcagatcacaaagcacgtggcacagatcctggactcccggatgaacactaagtacgacgagaatgacaagctgatccgggaagtgaaagtgatcaccctgaagtccaagctggtgtccgatttccggaaggatttccagttttacaaagtgcgcgagatcaacaactaccaccacgcccacgacgcctacctgaacgccgtcgtgggaaccgccctgatcaaaaagtaccctaagctggaaagcgagttcgtgtacggcgactacaaggtgtacgacgtgcggaagatgatcgccaagagcgagcaggaaatcggcaaggctaccgccaagtacttcttctacagcaacatcatgaactttttcaagaccgagattaccctggccaacggcgagatccggaagcggcctctgatcgagacaaacggcgaaaccggggagatcgtgtgggataagggccgggattttgccaccgtgcggaaagtgctgagcatgccccaagtgaatatcgtgaaaaagaccgaggtgcagacaggcggcttcagcaaagagtctatcctgcccaagaggaacagcgataagctgatcgccagaaagaaggactgggaccctaagaagtacggcggcttcgacagccccaccgtggcctattctgtgctggtggtggccaaagtggaaaagggcaagtccaagaaactgaagagtgtgaaagagctgctggggatcaccatcatggaaagaagcagcttcgagaagaatcccatcgactttctggaagccaagggctacaaagaagtgaaaaaggacctgatcatcaagctgcctaagtactccctgttcgagctggaaaacggccggaagagaatgctggcctctgccggcgaactgcagaagggaaacgaactggccctgccctccaaatatgtgaacttcctgtacctggccagccactatgagaagctgaagggctcccccgaggataatgagcagaaacagctgtttgtggaacagcacaagcactacctggacgagatcatcgagcagatcagcgagttctccaagagagtgatcctggccgacgctaatctggacaaagtgctgtccgcctacaacaagcaccgggataagcccatcagagagcaggccgagaatatcatccacctgtttaccctgaccaatctgggagcccctgccgccttcaagtactttgacaccaccatcgaccggaagaggtacaccagcaccaaagaggtgctggacgccaccctgatccaccagagcatcaccggcctgtacgagacacggatcgacctgtctcagctgggaggtgactctggcggctcaaaaagaaccgccgacggcagcgaattcgagcccaagaagaagaggaaagtc

SEQ ID NO: 160 - DNA, 4857 bp, synthetic construct
  source 1..4857: mol_type = other DNA
atgaaacggacagccgacggaagcgagttcgagtcaccaaagaagaagcggaaagtcatgtacaatgcccctagattcttttgtagatctgctgccgtgtctgatcatgagtttaacgatgagtactggatgagacacgccctgacactggccagaaagtctcgggaggaaggagaggtgccagtgggagctgtgctggtgctgaataatcaggtcattggagaaggatggaatagagccatcggcctgcacgaccccaccgcccacgccgagatcatggccctgagacagggcggcctggtgctgcagaactaccggctgatcgacgccaccctgtacgtgaccttcgagccctgcgtgatgtgcgccggcgccatggtgcatagcagaatcagcagactggtgttcggcgtgagaaactcaaagagaggcgccgccggcagcctgatcaacgtgctgaactaccccggcatgaaccacagagtggagatcaccgagggcatcctggccgagagctgcagcgccatgctgtgcgacttctataggtggcctagggaggtgttcaatgccctgaagaaggccagacaggaggagggctccggaggatctagcggaggctcctctggctctgagacacctggcacaagcgagagcgcaacacctgaaagcagcgggggcagcagcggggggtcagacaagaagtacagcatcggcctggccatcggcaccaactctgtgggctgggccgtgatcaccgacgagtacaaggtgcccagcaagaaattcaaggtgctgggcaacaccgaccggcacagcatcaagaagaacctgatcggagccctgctgttcgacagcggcgaaacagccgaggccacccggctgaagagaaccgccagaagaagatacaccagacggaagaaccggatctgctatctgcaagagatcttcagcaacgagatggccaaggtggacgacagcttcttccacagactggaagagtccttcctggtggaagaggataagaagcacgagcggcaccccatcttcggcaacatcgtggacgaggtggcctaccacgagaagtaccccaccatctaccacctgagaaagaaactggtggacagcaccgacaaggccgacctgcggctgatctatctggccctggcccacatgatcaagttccggggccacttcctgatcgagggcgacctgaaccccgacaacagcgacgtggacaagctgttcatccagctggtgcagacctacaaccagctgttcgaggaaaaccccatcaacgccagcggcgtggacgccaaggccatcctgtctgccagactgagcaagagcagacggctggaaaatctgatcgcccagctgcccggcgagaagaagaatggcctgttcggaaacctgattgccctgagcctgggcctgacccccaacttcaagagcaacttcgacctggccgaggatgccaaactgcagctgagcaaggacacctacgacgacgacctggacaacctgctggcccagatcggcgaccagtacgccgacctgtttctggccgccaagaacctgtccgacgccatcctgctgagcgacatcctgagagtgaacaccgagatcaccaaggcccccctgagcgcctctatgatcaagagatacgacgagcaccaccaggacctgaccctgctgaaagctctcgtgcggcagcagctgcctgagaagtacaaagagattttcttcgaccagagcaagaacggctacgccggctacattgacggcggagccagccaggaagagttctacaagttcatcaagcccatcctggaaaagatggacggcaccgaggaactgctcgtgaagctgaacagagaggacctgctgcggaagcagcggaccttcgacaacggcagcatcccccaccagatccacctgggagagctgcacgccattctgcggcggcaggaagatttttacccattcctgaaggacaaccgggaaaagatcgagaagatcctgaccttccgcatcccctactacgtgggccctctggccaggggaaacagcagattcgcctggatgaccagaaagagcgaggaaaccatcaccccctggaacttcgaggaagtggtggacaagggcgcttccgcccagagcttcatcgagcggatgaccaacttcgataagaacctgcccaacgagaaggtgctgcccaagcacagcctgctgtacgagtacttcaccgtgtataacgagctgaccaaagtgaaatacgtgaccgagggaatgagaaagcccgccttcctgagcggcgagcagaaaaaggccatcgtggacctgctgttcaagaccaaccggaaagtgaccgtgaagcagctgaaagaggactacttcaagaaaatcgagtgcttcgactccgtggaaatctccggcgtggaagatcggttcaacgcctccctgggcacataccacgatctgctgaaaattatcaaggacaaggacttcctggacaatgaggaaaacgaggacattctggaagatatcgtgctgaccctgacactgtttgaggacagagagatgatcgaggaacggctgaaaacctatgcccacctgttcgacgacaaagtgatgaagcagctgaagcggcggagatacaccggctggggcaggctgagccggaagctgatcaacggcatccgggacaagcagtccggcaagacaatcctggatttcctgaagtccgacggcttcgccaacagaaacttcatgcagctgatccacgacgacagcctgacctttaaagaggacatccagaaagcccaggtgtccggccagggcgatagcctgcacgagcacattgccaatctggccggcagccccgccattaagaagggcatcctgcagacagtgaaggtggtggacgagctcgtgaaagtgatgggccggcacaagcccgagaacatcgtgatcgaaatggccagagagaaccagaccacccagaagggacagaagaacagccgcgagagaatgaagcggatcgaagagggcatcaaagagctgggcagccagatcctgaaagaacaccccgtggaaaacacccagctgcagaacgagaagctgtacctgtactacctgcagaatgggcgggatatgtacgtggaccaggaactggacatcaaccggctgtccgactacgatgtggaccatatcgtgcctcagagctttctgaaggacgactccatcgacaacaaggtgctgaccagaagcgacaagaaccggggcaagagcgacaacgtgccctccgaagaggtcgtgaagaagatgaagaactactggcggcagctgctgaacgccaagctgattacccagagaaagttcgacaatctgaccaaggccgagagaggcggcctgagcgaactggataaggccggcttcatcaagagacagctggtggaaacccggcagatcacaaagcacgtggcacagatcctggactcccggatgaacactaagtacgacgagaatgacaagctgatccgggaagtgaaagtgatcaccctgaagtccaagctggtgtccgatttccggaaggatttccagttttacaaagtgcgcgagatcaacaactaccaccacgcccacgacgcctacctgaacgccgtcgtgggaaccgccctgatcaaaaagtaccctaagctggaaagcgagttcgtgtacggcgactacaaggtgtacgacgtgcggaagatgatcgccaagagcgagcaggaaatcggcaaggctaccgccaagtacttcttctacagcaacatcatgaactttttcaagaccgagattaccctggccaacggcgagatccggaagcggcctctgatcgagacaaacggcgaaaccggggagatcgtgtgggataagggccgggattttgccaccgtgcggaaagtgctgagcatgccccaagtgaatatcgtgaaaaagaccgaggtgcagacaggcggcttcagcaaagagtctatcctgcccaagaggaacagcgataagctgatcgccagaaagaaggactgggaccctaagaagtacggcggcttcgacagccccaccgtggcctattctgtgctggtggtggccaaagtggaaaagggcaagtccaagaaactgaagagtgtgaaagagctgctggggatcaccatcatggaaagaagcagcttcgagaagaatcccatcgactttctggaagccaagggctacaaagaagtgaaaaaggacctgatcatcaagctgcctaagtactccctgttcgagctggaaaacggccggaagagaatgctggcctctgccggcgaactgcagaagggaaacgaactggccctgccctccaaatatgtgaacttcctgtacctggccagccactatgagaagctgaagggctcccccgaggataatgagcagaaacagctgtttgtggaacagcacaagcactacctggacgagatcatcgagcagatcagcgagttctccaagagagtgatcctggccgacgctaatctggacaaagtgctgtccgcctacaacaagcaccgggataagcccatcagagagcaggccgagaatatcatccacctgtttaccctgaccaatctgggagcccctgccgccttcaagtactttgacaccaccatcgaccggaagaggtacaccagcaccaaagaggtgctggacgccaccctgatccaccagagcatcaccggcctgtacgagacacggatcgacctgtctcagctgggaggtgactctggcggctcaaaaagaaccgccgacggcagcgaattcgagcccaagaagaagaggaaagtc

SEQ ID NO: 161 - DNA, 4857 bp, synthetic construct
  source 1..4857: mol_type = other DNA
atgaaacggacagccgacggaagcgagttcgagtcaccaaagaagaagcggaaagtcatgtacaatgcccctagattcttttgtagatctgctgccgtgtctgatcatgagtttaacgatgagtactggatgagacacgccctgacactggccaagagggctcgggaggaaggagaggtgccagtgggagctgtgctggtgctgaataatcaggtcattggagaaggatggaatagagccatcggcctgcacgaccccaccgcccacgccgagatcatggccctgagacagggcgccaatgccattaacagctggcggctgatcgacgccaccctgtacgtgaccttcgagccctgcgtgatgtgcgccggcgccatggtgcatagcagaatcagcagactggtgttcggcgtgagaaactcaaagagaggcgccgccggcagcctgatcaacgtgctgaactaccccggcatgaaccacagagtggagatcaccgagggcatcctggccgagagctgcagcgccatgctgtgcgacttctataggtggcctagggaggtgttcaatgccctgaagaaggccagacaggaggagggctccggaggatctagcggaggctcctctggctctgagacacctggcacaagcgagagcgcaacacctgaaagcagcgggggcagcagcggggggtcagacaagaagtacagcatcggcctggccatcggcaccaactctgtgggctgggccgtgatcaccgacgagtacaaggtgcccagcaagaaattcaaggtgctgggcaacaccgaccggcacagcatcaagaagaacctgatcggagccctgctgttcgacagcggcgaaacagccgaggccacccggctgaagagaaccgccagaagaagatacaccagacggaagaaccggatctgctatctgcaagagatcttcagcaacgagatggccaaggtggacgacagcttcttccacagactggaagagtccttcctggtggaagaggataagaagcacgagcggcaccccatcttcggcaacatcgtggacgaggtggcctaccacgagaagtaccccaccatctaccacctgagaaagaaactggtggacagcaccgacaaggccgacctgcggctgatctatctggccctggcccacatgatcaagttccggggccacttcctgatcgagggcgacctgaaccccgacaacagcgacgtggacaagctgttcatccagctggtgcagacctacaaccagctgttcgaggaaaaccccatcaacgccagcggcgtggacgccaaggccatcctgtctgccagactgagcaagagcagacggctggaaaatctgatcgcccagctgcccggcgagaagaagaatggcctgttcggaaacctgattgccctgagcctgggcctgacccccaacttcaagagcaacttcgacctggccgaggatgccaaactgcagctgagcaaggacacctacgacgacgacctggacaacctgctggcccagatcggcgaccagtacgccgacctgtttctggccgccaagaacctgtccgacgccatcctgctgagcgacatcctgagagtgaacaccgagatcaccaaggcccccctgagcgcctctatgatcaagagatacgacgagcaccaccaggacctgaccctgctgaaagctctcgtgcggcagcagctgcctgagaagtacaaagagattttcttcgaccagagcaagaacggctacgccggctacattgacggcggagccagccaggaagagttctacaagttcatcaagcccatcctggaaaagatggacggcaccgaggaactgctcgtgaagctgaacagagaggacctgctgcggaagcagcggaccttcgacaacggcagcatcccccaccagatccacctgggagagctgcacgccattctgcggcggcaggaagatttttacccattcctgaaggacaaccgggaaaagatcgagaagatcctgaccttccgcatcccctactacgtgggccctctggccaggggaaacagcagattcgcctggatgaccagaaagagcgaggaaaccatcaccccctggaacttcgaggaagtggtggacaagggcgcttccgcccagagcttcatcgagcggatgaccaacttcgataagaacctgcccaacgagaaggtgctgcccaagcacagcctgctgtacgagtacttcaccgtgtataacgagctgaccaaagtgaaatacgtgaccgagggaatgagaaagcccgccttcctgagcggcgagcagaaaaaggccatcgtggacctgctgttcaagaccaaccggaaagtgaccgtgaagcagctgaaagaggactacttcaagaaaatcgagtgcttcgactccgtggaaatctccggcgtggaagatcggttcaacgcctccctgggcacataccacgatctgctgaaaattatcaaggacaaggacttcctggacaatgaggaaaacgaggacattctggaagatatcgtgctgaccctgacactgtttgaggacagagagatgatcgaggaacggctgaaaacctatgcccacctgttcgacgacaaagtgatgaagcagctgaagcggcggagatacaccggctggggcaggctgagccggaagctgatcaacggcatccgggacaagcagtccggcaagacaatcctggatttcctgaagtccgacggcttcgccaacagaaacttcatgcagctgatccacgacgacagcctgacctttaaagaggacatccagaaagcccaggtgtccggccagggcgatagcctgcacgagcacattgccaatctggccggcagccccgccattaagaagggcatcctgcagacagtgaaggtggtggacgagctcgtgaaagtgatgggccggcacaagcccgagaacatcgtgatcgaaatggccagagagaaccagaccacccagaagggacagaagaacagccgcgagagaatgaagcggatcgaagagggcatcaaagagctgggcagccagatcctgaaagaacaccccgtggaaaacacccagctgcagaacgagaagctgtacctgtactacctgcagaatgggcgggatatgtacgtggaccaggaactggacatcaaccggctgtccgactacgatgtggaccatatcgtgcctcagagctttctgaaggacgactccatcgacaacaaggtgctgaccagaagcgacaagaaccggggcaagagcgacaacgtgccctccgaagaggtcgtgaagaagatgaagaactactggcggcagctgctgaacgccaagctgattacccagagaaagttcgacaatctgaccaaggccgagagaggcggcctgagcgaactggataaggccggcttcatcaagagacagctggtggaaacccggcagatcacaaagcacgtggcacagatcctggactcccggatgaacactaagtacgacgagaatgacaagctgatccgggaagtgaaagtgatcaccctgaagtccaagctggtgtccgatttccggaaggatttccagttttacaaagtgcgcgagatcaacaactaccaccacgcccacgacgcctacctgaacgccgtcgtgggaaccgccctgatcaaaaagtaccctaagctggaaagcgagttcgtgtacggcgactacaaggtgtacgacgtgcggaagatgatcgccaagagcgagcaggaaatcggcaaggctaccgccaagtacttcttctacagcaacatcatgaactttttcaagaccgagattaccctggccaacggcgagatccggaagcggcctctgatcgagacaaacggcgaaaccggggagatcgtgtgggataagggccgggattttgccaccgtgcggaaagtgctgagcatgccccaagtgaatatcgtgaaaaagaccgaggtgcagacaggcggcttcagcaaagagtctatcctgcccaagaggaacagcgataagctgatcgccagaaagaaggactgggaccctaagaagtacggcggcttcgacagccccaccgtggcctattctgtgctggtggtggccaaagtggaaaagggcaagtccaagaaactgaagagtgtgaaagagctgctggggatcaccatcatggaaagaagcagcttcgagaagaatcccatcgactttctggaagccaagggctacaaagaagtgaaaaaggacctgatcatcaagctgcctaagtactccctgttcgagctggaaaacggccggaagagaatgctggcctctgccggcgaactgcagaagggaaacgaactggccctgccctccaaatatgtgaacttcctgtacctggccagccactatgagaagctgaagggctcccccgaggataatgagcagaaacagctgtttgtggaacagcacaagcactacctggacgagatcatcgagcagatcagcgagttctccaagagagtgatcctggccgacgctaatctggacaaagtgctgtccgcctacaacaagcaccgggataagcccatcagagagcaggccgagaatatcatccacctgtttaccctgaccaatctgggagcccctgccgccttcaagtactttgacaccaccatcgaccggaagaggtacaccagcaccaaagaggtgctggacgccaccctgatccaccagagcatcaccggcctgtacgagacacggatcgacctgtctcagctgggaggtgactctggcggctcaaaaagaaccgccgacggcagcgaattcgagcccaagaagaagaggaaagtc

SEQ ID NO: 162 - DNA, 4857 bp, synthetic construct
  source 1..4857: mol_type = other DNA
atgaaacggacagccgacggaagcgagttcgagtcaccaaagaagaagcggaaagtcatgtacaatgcccctagattcttttgtagatctgctgccgtgtctgatcatgagtttaacgatgagtactggatgagacacgccctgacactggccaagagggctcgggaggaaggagaggtgccagtgggagctgtgctggtgctgaataatcaggtcattggagaaggatggaatagagccatcggcctgcacgaccccaccgcccacgccgagatcatggccctgagacagggcggcctggtgctgcagaactaccggctgctgggaacagacctgtacgtgaccttcgagccctgcgtgatgtgcgccggcgccatggtgcatagcagaatcagcagactggtgttcggcgtgagaaactcaaagagaggcgccgccggcagcctgatcaacgtgctgaactaccccggcatgaaccacagagtggagatcaccgagggcatcctggccgagagctgcagcgccatgctgtgcgacttctataggtggcctagggaggtgttcaatgccctgaagaaggccagacaggaggagggctccggaggatctagcggaggctcctctggctctgagacacctggcacaagcgagagcgcaacacctgaaagcagcgggggcagcagcggggggtcagacaagaagtacagcatcggcctggccatcggcaccaactctgtgggctgggccgtgatcaccgacgagtacaaggtgcccagcaagaaattcaaggtgctgggcaacaccgaccggcacagcatcaagaagaacctgatcggagccctgctgttcgacagcggcgaaacagccgaggccacccggctgaagagaaccgccagaagaagatacaccagacggaagaaccggatctgctatctgcaagagatcttcagcaacgagatggccaaggtggacgacagcttcttccacagactggaagagtccttcctggtggaagaggataagaagcacgagcggcaccccatcttcggcaacatcgtggacgaggtggcctaccacgagaagtaccccaccatctaccacctgagaaagaaactggtggacagcaccgacaaggccgacctgcggctgatctatctggccctggcccacatgatcaagttccggggccacttcctgatcgagggcgacctgaaccccgacaacagcgacgtggacaagctgttcatccagctggtgcagacctacaaccagctgttcgaggaaaaccccatcaacgccagcggcgtggacgccaaggccatcctgtctgccagactgagcaagagcagacggctggaaaatctgatcgcccagctgcccggcgagaagaagaatggcctgttcggaaacctgattgccctgagcctgggcctgacccccaacttcaagagcaacttcgacctggccgaggatgccaaactgcagctgagcaaggacacctacgacgacgacctggacaacctgctggcccagatcggcgaccagtacgccgacctgtttctggccgccaagaacctgtccgacgccatcctgctgagcgacatcctgagagtgaacaccgagatcaccaaggcccccctgagcgcctctatgatcaagagatacgacgagcaccaccaggacctgaccctgctgaaagctctcgtgcggcagcagctgcctgagaagtacaaagagattttcttcgaccagagcaagaacggctacgccggctacattgacggcggagccagccaggaagagttctacaagttcatcaagcccatcctggaaaagatggacggcaccgaggaactgctcgtgaagctgaacagagaggacctgctgcggaagcagcggaccttcgacaacggcagcatcccccaccagatccacctgggagagctgcacgccattctgcggcggcaggaagatttttacccattcctgaaggacaaccgggaaaagatcgagaagatcctgaccttccgcatcccctactacgtgggccctctggccaggggaaacagcagattcgcctggatgaccagaaagagcgaggaaaccatcaccccctggaacttcgaggaagtggtggacaagggcgcttccgcccagagcttcatcgagcggatgaccaacttcgataagaacctgcccaacgagaaggtgctgcccaagcacagcctgctgtacgagtacttcaccgtgtataacgagctgaccaaagtgaaatacgtgaccgagggaatgagaaagcccgccttcctgagcggcgagcagaaaaaggccatcgtggacctgctgttcaagaccaaccggaaagtgaccgtgaagcagctgaaagaggactacttcaagaaaatcgagtgcttcgactccgtggaaatctccggcgtggaagatcggttcaacgcctccctgggcacataccacgatctgctgaaaattatcaaggacaaggacttcctggacaatgaggaaaacgaggacattctggaagatatcgtgctgaccctgacactgtttgaggacagagagatgatcgaggaacggctgaaaacctatgcccacctgttcgacgacaaagtgatgaagcagctgaagcggcggagatacaccggctggggcaggctgagccggaagctgatcaacggcatccgggacaagcagtccggcaagacaatcctggatttcctgaagtccgacggcttcgccaacagaaacttcatgcagctgatccacgacgacagcctgacctttaaagaggacatccagaaagcccaggtgtccggccagggcgatagcctgcacgagcacattgccaatctggccggcagccccgccattaagaagggcatcctgcagacagtgaaggtggtggacgagctcgtgaaagtgatgggccggcacaagcccgagaacatcgtgatcgaaatggccagagagaaccagaccacccagaagggacagaagaacagccgcgagagaatgaagcggatcgaagagggcatcaaagagctgggcagccagatcctgaaagaacaccccgtggaaaacacccagctgcagaacgagaagctgtacctgtactacctgcagaatgggcgggatatgtacgtggaccaggaactggacatcaaccggctgtccgactacgatgtggaccatatcgtgcctcagagctttctgaaggacgactccatcgacaacaaggtgctgaccagaagcgacaagaaccggggcaagagcgacaacgtgccctccgaagaggtcgtgaagaagatgaagaactactggcggcagctgctgaacgccaagctgattacccagagaaagttcgacaatctgaccaaggccgagagaggcggcctgagcgaactggataaggccggcttcatcaagagacagctggtggaaacccggcagatcacaaagcacgtggcacagatcctggactcccggatgaacactaagtacgacgagaatgacaagctgatccgggaagtgaaagtgatcaccctgaagtccaagctggtgtccgatttccggaaggatttccagttttacaaagtgcgcgagatcaacaactaccaccacgcccacgacgcctacctgaacgccgtcgtgggaaccgccctgatcaaaaagtaccctaagctggaaagcgagttcgtgtacggcgactacaaggtgtacgacgtgcggaagatgatcgccaagagcgagcaggaaatcggcaaggctaccgccaagtacttcttctacagcaacatcatgaactttttcaagaccgagattaccctggccaacggcgagatccggaagcggcctctgatcgagacaaacggcgaaaccggggagatcgtgtgggataagggccgggattttgccaccgtgcggaaagtgctgagcatgccccaagtgaatatcgtgaaaaagaccgaggtgcagacaggcggcttcagcaaagagtctatcctgcccaagaggaacagcgataagctgatcgccagaaagaaggactgggaccctaagaagtacggcggcttcgacagccccaccgtggcctattctgtgctggtggtggccaaagtggaaaagggcaagtccaagaaactgaagagtgtgaaagagctgctggggatcaccatcatggaaagaagcagcttcgagaagaatcccatcgactttctggaagccaagggctacaaagaagtgaaaaaggacctgatcatcaagctgcctaagtactccctgttcgagctggaaaacggccggaagagaatgctggcctctgccggcgaactgcagaagggaaacgaactggccctgccctccaaatatgtgaacttcctgtacctggccagccactatgagaagctgaagggctcccccgaggataatgagcagaaacagctgtttgtggaacagcacaagcactacctggacgagatcatcgagcagatcagcgagttctccaagagagtgatcctggccgacgctaatctggacaaagtgctgtccgcctacaacaagcaccgggataagcccatcagagagcaggccgagaatatcatccacctgtttaccctgaccaatctgggagcccctgccgccttcaagtactttgacaccaccatcgaccggaagaggtacaccagcaccaaagaggtgctggacgccaccctgatccaccagagcatcaccggcctgtacgagacacggatcgacctgtctcagctgggaggtgactctggcggctcaaaaagaaccgccgacggcagcgaattcgagcccaagaagaagaggaaagtc

SEQ ID NO: 163 - DNA, 4857 bp, synthetic construct
  source 1..4857: mol_type = other DNA
atgaaacggacagccgacggaagcgagttcgagtcaccaaagaagaagcggaaagtcatgtacaatgcccctagattcttttgtagatctgctgccgtgtctgatcatgagtttaacgatgagtactggatgagacacgccctgacactggccaagagggctcgggaggaaggagaggtgccagtgggagctgtgctggtgctgaataatcaggtcattggagaaggatggaatagagccatcggcctgcacgaccccaccgcccacgccgagatcatggccctgagacagggcggcctggtgctgcagaactaccggctgatcgacgccaccctgtacgtgaccttcgagccctgcgtgatgtgcgccggcgccatggtgcatagcagattgaagaaactggtgttcggcgtgagaaactcaaagagaggcgccgccggcagcctgatcaacgtgctgaactaccccggcatgaaccacagagtggagatcaccgagggcatcctggccgagagctgcagcgccatgctgtgcgacttctataggtggcctagggaggtgttcaatgccctgaagaaggccagacaggaggagggctccggaggatctagcggaggctcctctggctctgagacacctggcacaagcgagagcgcaacacctgaaagcagcgggggcagcagcggggggtcagacaagaagtacagcatcggcctggccatcggcaccaactctgtgggctgggccgtgatcaccgacgagtacaaggtgcccagcaagaaattcaaggtgctgggcaacaccgaccggcacagcatcaagaagaacctgatcggagccctgctgttcgacagcggcgaaacagccgaggccacccggctgaagagaaccgccagaagaagatacaccagacggaagaaccggatctgctatctgcaagagatcttcagcaacgagatggccaaggtggacgacagcttcttccacagactggaagagtccttcctggtggaagaggataagaagcacgagcggcaccccatcttcggcaacatcgtggacgaggtggcctaccacgagaagtaccccaccatctaccacctgagaaagaaactggtggacagcaccgacaaggccgacctgcggctgatctatctggccctggcccacatgatcaagttccggggccacttcctgatcgagggcgacctgaaccccgacaacagcgacgtggacaagctgttcatccagctggtgcagacctacaaccagctgttcgaggaaaaccccatcaacgccagcggcgtggacgccaaggccatcctgtctgccagactgagcaagagcagacggctggaaaatctgatcgcccagctgcccggcgagaagaagaatggcctgttcggaaacctgattgccctgagcctgggcctgacccccaacttcaagagcaacttcgacctggccgaggatgccaaactgcagctgagcaaggacacctacgacgacgacctggacaacctgctggcccagatcggcgaccagtacgccgacctgtttctggccgccaagaacctgtccgacgccatcctgctgagcgacatcctgagagtgaacaccgagatcaccaaggcccccctgagcgcctctatgatcaagagatacgacgagcaccaccaggacctgaccctgctgaaagctctcgtgcggcagcagctgcctgagaagtacaaagagattttcttcgaccagagcaagaacggctacgccggctacattgacggcggagccagccaggaagagttctacaagttcatcaagcccatcctggaaaagatggacggcaccgaggaactgctcgtgaagctgaacagagaggacctgctgcggaagcagcggaccttcgacaacggcagcatcccccaccagatccacctgggagagctgcacgccattctgcggcggcaggaagatttttacccattcctgaaggacaaccgggaaaagatcgagaagatcctgaccttccgcatcccctactacgtgggccctctggccaggggaaacagcagattcgcctggatgaccagaaagagcgaggaaaccatcaccccctggaacttcgaggaagtggtggacaagggcgcttccgcccagagcttcatcgagcggatgaccaacttcgataagaacctgcccaacgagaaggtgctgcccaagcacagcctgctgtacgagtacttcaccgtgtataacgagctgaccaaagtgaaatacgtgaccgagggaatgagaaagcccgccttcctgagcggcgagcagaaaaaggccatcgtggacctgctgttcaagaccaaccggaaagtgaccgtgaagcagctgaaagaggactacttcaagaaaatcgagtgcttcgactccgtggaaatctccggcgtggaagatcggttcaacgcctccctgggcacataccacgatctgctgaaaattatcaaggacaaggacttcctggacaatgaggaaaacgaggacattctggaagatatcgtgctgaccctgacactgtttgaggacagagagatgatcgaggaacggctgaaaacctatgcccacctgttcgacgacaaagtgatgaagcagctgaagcggcggagatacaccggctggggcaggctgagccggaagctgatcaacggcatccgggacaagcagtccggcaagacaatcctggatttcctgaagtccgacggcttcgccaacagaaacttcatgcagctgatccacgacgacagcctgacctttaaagaggacatccagaaagcccaggtgtccggccagggcgatagcctgcacgagcacattgccaatctggccggcagccccgccattaagaagggcatcctgcagacagtgaaggtggtggacgagctcgtgaaagtgatgggccggcacaagcccgagaacatcgtgatcgaaatggccagagagaaccagaccacccagaagggacagaagaacagccgcgagagaatgaagcggatcgaagagggcatcaaagagctgggcagccagatcctgaaagaacaccccgtggaaaacacccagctgcagaacgagaagctgtacctgtactacctgcagaatgggcgggatatgtacgtggaccaggaactggacatcaaccggctgtccgactacgatgtggaccatatcgtgcctcagagctttctgaaggacgactccatcgacaacaaggtgctgaccagaagcgacaagaaccggggcaagagcgacaacgtgccctccgaagaggtcgtgaagaagatgaagaactactggcggcagctgctgaacgccaagctgattacccagagaaagttcgacaatctgaccaaggccgagagaggcggcctgagcgaactggataaggccggcttcatcaagagacagctggtggaaacccggcagatcacaaagcacgtggcacagatcctggactcccggatgaacactaagtacgacgagaatgacaagctgatccgggaagtgaaagtgatcaccctgaagtccaagctggtgtccgatttccggaaggatttccagttttacaaagtgcgcgagatcaacaactaccaccacgcccacgacgcctacctgaacgccgtcgtgggaaccgccctgatcaaaaagtaccctaagctggaaagcgagttcgtgtacggcgactacaaggtgtacgacgtgcggaagatgatcgccaagagcgagcaggaaatcggcaaggctaccgccaagtacttcttctacagcaacatcatgaactttttcaagaccgagattaccctggccaacggcgagatccggaagcggcctctgatcgagacaaacggcgaaaccggggagatcgtgtgggataagggccgggattttgccaccgtgcggaaagtgctgagcatgccccaagtgaatatcgtgaaaaagaccgaggtgcagacaggcggcttcagcaaagagtctatcctgcccaagaggaacagcgataagctgatcgccagaaagaaggactgggaccctaagaagtacggcggcttcgacagccccaccgtggcctattctgtgctggtggtggccaaagtggaaaagggcaagtccaagaaactgaagagtgtgaaagagctgctggggatcaccatcatggaaagaagcagcttcgagaagaatcccatcgactttctggaagccaagggctacaaagaagtgaaaaaggacctgatcatcaagctgcctaagtactccctgttcgagctggaaaacggccggaagagaatgctggcctctgccggcgaactgcagaagggaaacgaactggccctgccctccaaatatgtgaacttcctgtacctggccagccactatgagaagctgaagggctcccccgaggataatgagcagaaacagctgtttgtggaacagcacaagcactacctggacgagatcatcgagcagatcagcgagttctccaagagagtgatcctggccgacgctaatctggacaaagtgctgtccgcctacaacaagcaccgggataagcccatcagagagcaggccgagaatatcatccacctgtttaccctgaccaatctgggagcccctgccgccttcaagtactttgacaccaccatcgaccggaagaggtacaccagcaccaaagaggtgctggacgccaccctgatccaccagagcatcaccggcctgtacgagacacggatcgacctgtctcagctgggaggtgactctggcggctcaaaaagaaccgccgacggcagcgaattcgagcccaagaagaagaggaaagtc

SEQ ID NO: 164 - DNA, 4857 bp, synthetic construct
  source 1..4857: mol_type = other DNA
atgaaacggacagccgacggaagcgagttcgagtcaccaaagaagaagcggaaagtcatgtacaatgcccctagattcttttgtagatctgctgccgtgtctgatcatgagtttaacgatgagtactggatgagacacgccctgacactggccaagagggctcgggaggaaggagaggtgccagtgggagctgtgctggtgctgaataatcaggtcattggagaaggatggaatagagccatcggcctgcacgaccccaccgcccacgccgagatcatggccctgagacagggcggcctggtgctgcagaactaccggctgatcgacgccaccctgtacgtgaccttcgagccctgcgtgatgtgcgccggcgccatggtgcatagcagaatcagcagactggtgttcggcgtgagaaactcaaagagaggcgccgccggcagcctgatcaagatcttccactaccccggcatgaaccacagagtggagatcaccgagggcatcctggccgagagctgcagcgccatgctgtgcgacttctataggtggcctagggaggtgttcaatgccctgaagaaggccagacaggaggagggctccggaggatctagcggaggctcctctggctctgagacacctggcacaagcgagagcgcaacacctgaaagcagcgggggcagcagcggggggtcagacaagaagtacagcatcggcctggccatcggcaccaactctgtgggctgggccgtgatcaccgacgagtacaaggtgcccagcaagaaattcaaggtgctgggcaacaccgaccggcacagcatcaagaagaacctgatcggagccctgctgttcgacagcggcgaaacagccgaggccacccggctgaagagaaccgccagaagaagatacaccagacggaagaaccggatctgctatctgcaagagatcttcagcaacgagatggccaaggtggacgacagcttcttccacagactggaagagtccttcctggtggaagaggataagaagcacgagcggcaccccatcttcggcaacatcgtggacgaggtggcctaccacgagaagtaccccaccatctaccacctgagaaagaaactggtggacagcaccgacaaggccgacctgcggctgatctatctggccctggcccacatgatcaagttccggggccacttcctgatcgagggcgacctgaaccccgacaacagcgacgtggacaagctgttcatccagctggtgcagacctacaaccagctgttcgaggaaaaccccatcaacgccagcggcgtggacgccaaggccatcctgtctgccagactgagcaagagcagacggctggaaaatctgatcgcccagctgcccggcgagaagaagaatggcctgttcggaaacctgattgccctgagcctgggcctgacccccaacttcaagagcaacttcgacctggccgaggatgccaaactgcagctgagcaaggacacctacgacgacgacctggacaacctgctggcccagatcggcgaccagtacgccgacctgtttctggccgccaagaacctgtccgacgccatcctgctgagcgacatcctgagagtgaacaccgagatcaccaaggcccccctgagcgcctctatgatcaagagatacgacgagcaccaccaggacctgaccctgctgaaagctctcgtgcggcagcagctgcctgagaagtacaaagagattttcttcgaccagagcaagaacggctacgccggctacattgacggcggagccagccaggaagagttctacaagttcatcaagcccatcctggaaaagatggacggcaccgaggaactgctcgtgaagctgaacagagaggacctgctgcggaagcagcggaccttcgacaacggcagcatcccccaccagatccacctgggagagctgcacgccattctgcggcggcaggaagatttttacccattcctgaaggacaaccgggaaaagatcgagaagatcctgaccttccgcatcccctactacgtgggccctctggccaggggaaacagcagattcgcctggatgaccagaaagagcgaggaaaccatcaccccctggaacttcgaggaagtggtggacaagggcgcttccgcccagagcttcatcgagcggatgaccaacttcgataagaacctgcccaacgagaaggtgctgcccaagcacagcctgctgtacgagtacttcaccgtgtataacgagctgaccaaagtgaaatacgtgaccgagggaatgagaaagcccgccttcctgagcggcgagcagaaaaaggccatcgtggacctgctgttcaagaccaaccggaaagtgaccgtgaagcagctgaaagaggactacttcaagaaaatcgagtgcttcgactccgtggaaatctccggcgtggaagatcggttcaacgcctccctgggcacataccacgatctgctgaaaattatcaaggacaaggacttcctggacaatgaggaaaacgaggacattctggaagatatcgtgctgaccctgacactgtttgaggacagagagatgatcgaggaacggctgaaaacctatgcccacctgttcgacgacaaagtgatgaagcagctgaagcggcggagatacaccggctggggcaggctgagccggaagctgatcaacggcatccgggacaagcagtccggcaagacaatcctggatttcctgaagtccgacggcttcgccaacagaaacttcatgcagctgatccacgacgacagcctgacctttaaagaggacatccagaaagcccaggtgtccggccagggcgatagcctgcacgagcacattgccaatctggccggcagccccgccattaagaagggcatcctgcagacagtgaaggtggtggacgagctcgtgaaagtgatgggccggcacaagcccgagaacatcgtgatcgaaatggccagagagaaccagaccacccagaagggacagaagaacagccgcgagagaatgaagcggatcgaagagggcatcaaagagctgggcagccagatcctgaaagaacaccccgtggaaaacacccagctgcagaacgagaagctgtacctgtactacctgcagaatgggcgggatatgtacgtggaccaggaactggacatcaaccggctgtccgactacgatgtggaccatatcgtgcctcagagctttctgaaggacgactccatcgacaacaaggtgctgaccagaagcgacaagaaccggggcaagagcgacaacgtgccctccgaagaggtcgtgaagaagatgaagaactactggcggcagctgctgaacgccaagctgattacccagagaaagttcgacaatctgaccaaggccgagagaggcggcctgagcgaactggataaggccggcttcatcaagagacagctggtggaaacccggcagatcacaaagcacgtggcacagatcctggactcccggatgaacactaagtacgacgagaatgacaagctgatccgggaagtgaaagtgatcaccctgaagtccaagctggtgtccgatttccggaaggatttccagttttacaaagtgcgcgagatcaacaactaccaccacgcccacgacgcctacctgaacgccgtcgtgggaaccgccctgatcaaaaagtaccctaagctggaaagcgagttcgtgtacggcgactacaaggtgtacgacgtgcggaagatgatcgccaagagcgagcaggaaatcggcaaggctaccgccaagtacttcttctacagcaacatcatgaactttttcaagaccgagattaccctggccaacggcgagatccggaagcggcctctgatcgagacaaacggcgaaaccggggagatcgtgtgggataagggccgggattttgccaccgtgcggaaagtgctgagcatgccccaagtgaatatcgtgaaaaagaccgaggtgcagacaggcggcttcagcaaagagtctatcctgcccaagaggaacagcgataagctgatcgccagaaagaaggactgggaccctaagaagtacggcggcttcgacagccccaccgtggcctattctgtgctggtggtggccaaagtggaaaagggcaagtccaagaaactgaagagtgtgaaagagctgctggggatcaccatcatggaaagaagcagcttcgagaagaatcccatcgactttctggaagccaagggctacaaagaagtgaaaaaggacctgatcatcaagctgcctaagtactccctgttcgagctggaaaacggccggaagagaatgctggcctctgccggcgaactgcagaagggaaacgaactggccctgccctccaaatatgtgaacttcctgtacctggccagccactatgagaagctgaagggctcccccgaggataatgagcagaaacagctgtttgtggaacagcacaagcactacctggacgagatcatcgagcagatcagcgagttctccaagagagtgatcctggccgacgctaatctggacaaagtgctgtccgcctacaacaagcaccgggataagcccatcagagagcaggccgagaatatcatccacctgtttaccctgaccaatctgggagcccctgccgccttcaagtactttgacaccaccatcgaccggaagaggtacaccagcaccaaagaggtgctggacgccaccctgatccaccagagcatcaccggcctgtacgagacacggatcgacctgtctcagctgggaggtgactctggcggctcaaaaagaaccgccgacggcagcgaattcgagcccaagaagaagaggaaagtc

SEQ ID NO: 165 - DNA, 4857 bp, synthetic construct
  source 1..4857: mol_type = other DNA
atgaaacggacagccgacggaagcgagttcgagtcaccaaagaagaagcggaaagtcatgtacaatgcccctagattcttttgtagatctgctgccgtgtctgatcatgagtttaacgatgagtactggatgagacacgccctgacactggccaagagggctcgggaggaaggagaggtgccagtgggagctgtgctggtgctgaataatcaggtcattggagaaggatggaatagagccatcggcctgcacgaccccaccgcccacgccgagatcatggccctgagacagggcggcctggtgctgcagaactaccggctgatcgacgccaccctgtacgtgaccttcgagccctgcgtgatgtgcgccggcgccatggtgcatagcagaatcagcagactggtgttcggcgtgagaaactcaaagagaggcgccgccggcagcctgatcaacgtgctgaactacttcgccctgaaccacagagtggagatcaccgagggcatcctggccgagagctgcagcgccatgctgtgcgacttctataggtggcctagggaggtgttcaatgccctgaagaaggccagacaggaggagggctccggaggatctagcggaggctcctctggctctgagacacctggcacaagcgagagcgcaacacctgaaagcagcgggggcagcagcggggggtcagacaagaagtacagcatcggcctggccatcggcaccaactctgtgggctgggccgtgatcaccgacgagtacaaggtgcccagcaagaaattcaaggtgctgggcaacaccgaccggcacagcatcaagaagaacctgatcggagccctgctgttcgacagcggcgaaacagccgaggccacccggctgaagagaaccgccagaagaagatacaccagacggaagaaccggatctgctatctgcaagagatcttcagcaacgagatggccaaggtggacgacagcttcttccacagactggaagagtccttcctggtggaagaggataagaagcacgagcggcaccccatcttcggcaacatcgtggacgaggtggcctaccacgagaagtaccccaccatctaccacctgagaaagaaactggtggacagcaccgacaaggccgacctgcggctgatctatctggccctggcccacatgatcaagttccggggccacttcctgatcgagggcgacctgaaccccgacaacagcgacgtggacaagctgttcatccagctggtgcagacctacaaccagctgttcgaggaaaaccccatcaacgccagcggcgtggacgccaaggccatcctgtctgccagactgagcaagagcagacggctggaaaatctgatcgcccagctgcccggcgagaagaagaatggcctgttcggaaacctgattgccctgagcctgggcctgacccccaacttcaagagcaacttcgacctggccgaggatgccaaactgcagctgagcaaggacacctacgacgacgacctggacaacctgctggcccagatcggcgaccagtacgccgacctgtttctggccgccaagaacctgtccgacgccatcctgctgagcgacatcctgagagtgaacaccgagatcaccaaggcccccctgagcgcctctatgatcaagagatacgacgagcaccaccaggacctgaccctgctgaaagctctcgtgcggcagcagctgcctgagaagtacaaagagattttcttcgaccagagcaagaacggctacgccggctacattgacggcggagccagccaggaagagttctacaagttcatcaagcccatcctggaaaagatggacggcaccgaggaactgctcgtgaagctgaacagagaggacctgctgcggaagcagcggaccttcgacaacggcagcatcccccaccagatccacctgggagagctgcacgccattctgcggcggcaggaagatttttacccattcctgaaggacaaccgggaaaagatcgagaagatcctgaccttccgcatcccctactacgtgggccctctggccaggggaaacagcagattcgcctggatgaccagaaagagcgaggaaaccatcaccccctggaacttcgaggaagtggtggacaagggcgcttccgcccagagcttcatcgagcggatgaccaacttcgataagaacctgcccaacgagaaggtgctgcccaagcacagcctgctgtacgagtacttcaccgtgtataacgagctgaccaaagtgaaatacgtgaccgagggaatgagaaagcccgccttcctgagcggcgagcagaaaaaggccatcgtggacctgctgttcaagaccaaccggaaagtgaccgtgaagcagctgaaagaggactacttcaagaaaatcgagtgcttcgactccgtggaaatctccggcgtggaagatcggttcaacgcctccctgggcacataccacgatctgctgaaaattatcaaggacaaggacttcctggacaatgaggaaaacgaggacattctggaagatatcgtgctgaccctgacactgtttgaggacagagagatgatcgaggaacggctgaaaacctatgcccacctgttcgacgacaaagtgatgaagcagctgaagcggcggagatacaccggctggggcaggctgagccggaagctgatcaacggcatccgggacaagcagtccggcaagacaatcctggatttcctgaagtccgacggcttcgccaacagaaacttcatgcagctgatccacgacgacagcctgacctttaaagaggacatccagaaagcccaggtgtccggccagggcgatagcctgcacgagcacattgccaatctggccggcagccccgccattaagaagggcatcctgcagacagtgaaggtggtggacgagctcgtgaaagtgatgggccggcacaagcccgagaacatcgtgatcgaaatggccagagagaaccagaccacccagaagggacagaagaacagccgcgagagaatgaagcggatcgaagagggcatcaaagagctgggcagccagatcctgaaagaacaccccgtggaaaacacccagctgcagaacgagaagctgtacctgtactacctgcagaatgggcgggatatgtacgtggaccaggaactggacatcaaccggctgtccgactacgatgtggaccatatcgtgcctcagagctttctgaaggacgactccatcgacaacaaggtgctgaccagaagcgacaagaaccggggcaagagcgacaacgtgccctccgaagaggtcgtgaagaagatgaagaactactggcggcagctgctgaacgccaagctgattacccagagaaagttcgacaatctgaccaaggccgagagaggcggcctgagcgaactggataaggccggcttcatcaagagacagctggtggaaacccggcagatcacaaagcacgtggcacagatcctggactcccggatgaacactaagtacgacgagaatgacaagctgatccgggaagtgaaagtgatcaccctgaagtccaagctggtgtccgatttccggaaggatttccagttttacaaagtgcgcgagatcaacaactaccaccacgcccacgacgcctacctgaacgccgtcgtgggaaccgccctgatcaaaaagtaccctaagctggaaagcgagttcgtgtacggcgactacaaggtgtacgacgtgcggaagatgatcgccaagagcgagcaggaaatcggcaaggctaccgccaagtacttcttctacagcaacatcatgaactttttcaagaccgagattaccctggccaacggcgagatccggaagcggcctctgatcgagacaaacggcgaaaccggggagatcgtgtgggataagggccgggattttgccaccgtgcggaaagtgctgagcatgccccaagtgaatatcgtgaaaaagaccgaggtgcagacaggcggcttcagcaaagagtctatcctgcccaagaggaacagcgataagctgatcgccagaaagaaggactgggaccctaagaagtacggcggcttcgacagccccaccgtggcctattctgtgctggtggtggccaaagtggaaaagggcaagtccaagaaactgaagagtgtgaaagagctgctggggatcaccatcatggaaagaagcagcttcgagaagaatcccatcgactttctggaagccaagggctacaaagaagtgaaaaaggacctgatcatcaagctgcctaagtactccctgttcgagctggaaaacggccggaagagaatgctggcctctgccggcgaactgcagaagggaaacgaactggccctgccctccaaatatgtgaacttcctgtacctggccagccactatgagaagctgaagggctcccccgaggataatgagcagaaacagctgtttgtggaacagcacaagcactacctggacgagatcatcgagcagatcagcgagttctccaagagagtgatcctggccgacgctaatctggacaaagtgctgtccgcctacaacaagcaccgggataagcccatcagagagcaggccgagaatatcatccacctgtttaccctgaccaatctgggagcccctgccgccttcaagtactttgacaccaccatcgaccggaagaggtacaccagcaccaaagaggtgctggacgccaccctgatccaccagagcatcaccggcctgtacgagacacggatcgacctgtctcagctgggaggtgactctggcggctcaaaaagaaccgccgacggcagcgaattcgagcccaagaagaagaggaaagtc

SEQ ID NO: 166 - DNA, 20 bp, synthetic construct
  source 1..20: mol_type = other DNA
ctggctgaccaagagtgaag

SEQ ID NO: 167 - DNA, 20 bp, synthetic construct
  source 1..20: mol_type = other DNA
aatgagcctctggtggagat

SEQ ID NO: 168 - DNA, 8318 bp, synthetic construct
  source 1..8318: mol_type = other DNA
tgagctgataccgctcgccgcagccgaacgaccgagcgcagcgagtcagtgagcgaggaagcggaagagcgcccaatacgcaaaccgcctctccccgcgcgttggccgattcattaatgcagctggcacgacaggtttcccgactggaaagcgggcagtgagcgcaacgcaattaatgtgagttagctcactcattaggcaccccaggctttacactttatgcttccggctcgtatgttgtgtggaattgtgagcggataacaatttcacacaggaaacagctatgaccatgattacgccaagcgcgcaattaaccctcactaaagggaacaaaagctggagctgcaagcttaatgtagtcttatgcaatactcttgtagtcttgcaacatggtaacgatgagttagcaacatgccttacaaggagagaaaaagcaccgtgcatgccgattggtggaagtaaggtggtacgatcgtgccttattaggaaggcaacagacgggtctgacatggattggacgaaccactgaattgccgcattgcagagatattgtatttaagtgcctagctcgatacataaacgggtctctctggttagaccagatctgagcctgggagctctctggctaactagggaacccactgcttaagcctcaataaagcttgccttgagtgcttcaagtagtgtgtgcccgtctgttgtgtgactctggtaactagagatccctcagacccttttagtcagtgtggaaaatctctagcagtggcgcccgaacagggacttgaaagcgaaagggaaaccagaggagctctctcgacgcaggactcggcttgctgaagcgcgcacggcaagaggcgaggggcggcgactggtgagtacgccaaaaattttgactagcggaggctagaaggagagagatgggtgcgagagcgtcagtattaagcgggggagaattagatcgcgatgggaaaaaattcggttaaggccagggggaaagaaaaaatataaattaaaacatatagtatgggcaagcagggagctagaacgattcgcagttaatcctggcctgttagaaacatcagaaggctgtagacaaatactgggacagctacaaccatcccttcagacaggatcagaagaacttagatcattatataatacagtagcaaccctctattgtgtgcatcaaaggatagagataaaagacaccaaggaagctttagacaagatagaggaagagcaaaacaaaagtaagaccaccgcacagcaagcggccgctgatcttcagacctggaggaggagatatgagggacaattggagaagtgaattatataaatataaagtagtaaaaattgaaccattaggagtagcacccaccaaggcaaagagaagagtggtgcagagagaaaaaagagcagtgggaataggagctttgttccttgggttcttgggagcagcaggaagcactatgggcgcagcgtcaatgacgctgacggtacaggccagacaattattgtctggtatagtgcagcagcagaacaatttgctgagggctattgaggcgcaacagcatctgttgcaactcacagtctggggcatcaagcagctccaggcaagaatcctggctgtggaaagatacctaaaggatcaacagctcctggggatttggggttgctctggaaaactcatttgcaccactgctgtgccttggaatgctagttggagtaataaatctctggaacagatttggaatcacacgacctggatggagtgggacagagaaattaacaattacacaagcttaatacactccttaattgaagaatcgcaaaaccagcaagaaaagaatgaacaagaattattggaattagataaatgggcaagtttgtggaattggtttaacataacaaattggctgtggtatataaaattattcataatgatagtaggaggcttggtaggtttaagaatagtttttgctgtactttctatagtgaatagagttaggcagggatattcaccattatcgtttcagacccacctcccaaccccgaggggacccagagagggcctatttcccatgattccttcatatttgcatatacgatacaaggctgttagagagataattagaattaatttgactgtaaacacaaagatattagtacaaaatacgtgacgtagaaagtaataatttcttgggtagtttgcagttttaaaattatgttttaaaatggactatcatatgcttaccgtaacttgaaagtatttcgatttcttggctttatatatcttgtggaaaggacgaaacaccggagacggacgtctctgttttagagctagaaatagcaagttaaaataaggctagtccgttatcaacttgaaaaagtggcaccgagtcggtgcttttttaagcttggcgtaactagatcttgagacaaatggcagtattcatccacaattttaaaagaaaaggggggattggggggtacagtgcaggggaaagaatagtagacataatagcaacagacatacaaactaaagaattacaaaaacaaattacaaaaattcaaaattttcgggtttattacagggacagcagagatccactttggcgccggctcgagggggcccgggtgcaaagatggataaagttttaaacagagaggaatctttgcagctaatggaccttctaggtcttgaaaggagtgggaattggctccggtgcccgtcagtgggcagagcgcacatcgcccacagtccccgagaagttggggggaggggtcggcaattgatccggtgcctagagaaggtggcgcggggtaaactgggaaagtgatgtcgtgtactggctccgcctttttcccgagggtgggggagaaccgtatataagtgcagtagtcgccgtgaacgttctttttcgcaacgggtttgccgccagaacacaggtaagtgccgtgtgtggttcccgcgggcctggcctctttacgggttatggcccttgcgtgccttgaattacttccacctggctgcagtacgtgattcttgatcccgagcttcgggttggaagtgggtgggagagttcgaggccttgcgcttaaggagccccttcgcctcgtgcttgagttgaggcctggcctgggcgctggggccgccgcgtgcgaatctggtggcaccttcgcgcctgtctcgctgctttcgataagtctctagccatttaaaatttttgatgacctgctgcgacgctttttttctggcaagatagtcttgtaaatgcgggccaagatctgcacactggtatttcggtttttggggccgcgggcggcgacggggcccgtgcgtcccagcgcacatgttcggcgaggcggggcctgcgagcgcggccaccgagaatcggacgggggtagtctcaagctggccggcctgctctggtgcctggcctcgcgccgccgtgtatcgccccgccctgggcggcaaggctggcccggtcggcaccagttgcgtgagcggaaagatggccgcttcccggccctgctgcagggagctcaaaatggaggacgcggcgctcgggagagcgggcgggtgagtcacccacacaaaggaaaagggcctttccgtcctcagccgtcgcttcatgtgactccacggagtaccgggcgccgtccaggcacctcgattagttctcgagcttttggagtacgtcgtctttaggttggggggaggggttttatgcgatggagtttccccacactgagtgggtggagactgaagttaggccagcttggcacttgatgtaattctccttggaatttgccctttttgagtttggatcttggttcattctcaagcctcagacagtggttcaaagtttttttcttccatttcaggtgtcgtgacgtacggccaccatgaccgagtacaagcccacggtgcgcctcgccacccgcgacgacgtccccagggccgtacgcaccctcgccgccgcgttcgccgactaccccgccacgcgccacaccgtcgatccggaccgccacatcgagcgggtcaccgagctgcaagaactcttcctcacgcgcgtcgggctcgacatcggcaaggtgtgggtcgcggacgacggcgccgccgtggcggtctggaccacgccggagagcgtcgaagcgggggcggtgttcgccgagatcggcccgcgcatggccgagttgagcggttcccggctggccgcgcagcaacagatggaaggcctcctggcgccgcaccggcccaaggagcccgcgtggttcctggccaccgtcggagtctcgcccgaccaccagggcaagggtctgggcagcgccgtcgtgctccccggagtggaggcggccgagcgcgccggggtgcccgccttcctggagacctccgcgccccgcaacctccccttctacgagcggctcggcttcaccgtcaccgccgacgtcgaggtgcccgaaggaccgcgcacctggtgcatgacccgcaagcccggtgcctgaacgcgttaagtcgacaatcaacctctggattacaaaatttgtgaaagattgactggtattcttaactatgttgctccttttacgctatgtggatacgctgctttaatgcctttgtatcatgctattgcttcccgtatggctttcattttctcctccttgtataaatcctggttgctgtctctttatgaggagttgtggcccgttgtcaggcaacgtggcgtggtgtgcactgtgtttgctgacgcaacccccactggttggggcattgccaccacctgtcagctcctttccgggactttcgctttccccctccctattgccacggcggaactcatcgccgcctgccttgcccgctgctggacaggggctcggctgttgggcactgacaattccgtggtgttgtcggggaaatcatcgtcctttccttggctgctcgcctgtgttgccacctggattctgcgcgggacgtccttctgctacgtcccttcggccctcaatccagcggaccttccttcccgcggcctgctgccggctctgcggcctcttccgcgtcttcgccttcgccctcagacgagtcggatctccctttgggccgcctccccgcgtcgactttaagaccaatgacttacaaggcagctgtagatcttagccactttttaaaagaaaaggggggactggaagggctaattcactcccaacgaagacaagatctgctttttgcttgtactgggtctctctggttagaccagatctgagcctgggagctctctggctaactagggaacccactgcttaagcctcaataaagcttgccttgagtgcttcaagtagtgtgtgcccgtctgttgtgtgactctggtaactagagatccctcagacccttttagtcagtgtggaaaatctctagcagtacgtatagtagttcatgtcatcttattattcagtatttataacttgcaaagaaatgaatatcagagagtgagaggaacttgtttattgcagcttataatggttacaaataaagcaatagcatcacaaatttcacaaataaagcatttttttcactgcattctagttgtggtttgtccaaactcatcaatgtatcttatcatgtctggctctagctatcccgcccctaactccgcccatcccgcccctaactccgcccagttccgcccattctccgccccatggctgactaattttttttatttatgcagaggccgaggccgcctcggcctctgagctattccagaagtagtgaggaggcttttttggaggcctagggacgtacccaattcgccctatagtgagtcgtattacgcgcgctcactggccgtcgttttacaacgtcgtgactgggaaaaccctggcgttacccaacttaatcgccttgcagcacatccccctttcgccagctggcgtaatagcgaagaggcccgcaccgatcgcccttcccaacagttgcgcagcctgaatggcgaatgggacgcgccctgtagcggcgcattaagcgcggcgggtgtggtggttacgcgcagcgtgaccgctacacttgccagcgccctagcgcccgctcctttcgctttcttcccttcctttctcgccacgttcgccggctttccccgtcaagctctaaatcgggggctccctttagggttccgatttagtgctttacggcacctcgaccccaaaaaacttgattagggtgatggttcacgtagtgggccatcgccctgatagacggtttttcgccctttgacgttggagtccacgttctttaatagtggactcttgttccaaactggaacaacactcaaccctatctcggtctattcttttgatttataagggattttgccgatttcggcctattggttaaaaaatgagctgatttaacaaaaatttaacgcgaattttaacaaaatattaacgcttacaatttaggtggcacttttcggggaaatgtgcgcggaacccctatttgtttatttttctaaatacattcaaatatgtatccgctcatgagacaataaccctgataaatgcttcaataatattgaaaaaggaagagtatgagtattcaacatttccgtgtcgcccttattcccttttttgcggcattttgccttcctgtttttgctcacccagaaacgctggtgaaagtaaaagatgctgaagatcagttgggtgcacgagtgggttacatcgaactggatctcaacagcggtaagatccttgagagttttcgccccgaagaacgttttccaatgatgagcacttttaaagttctgctatgtggcgcggtattatcccgtattgacgccgggcaagagcaactcggtcgccgcatacactattctcagaatgacttggttgagtactcaccagtcacagaaaagcatcttacggatggcatgacagtaagagaattatgcagtgctgccataaccatgagtgataacactgcggccaacttacttctgacaacgatcggaggaccgaaggagctaaccgcttttttgcacaacatgggggatcatgtaactcgccttgatcgttgggaaccggagctgaatgaagccataccaaacgacgagcgtgacaccacgatgcctgtagcaatggcaacaacgttgcgcaaactattaactggcgaactacttactctagcttcccggcaacaattaatagactggatggaggcggataaagttgcaggaccacttctgcgctcggcccttccggctggctggtttattgctgataaatctggagccggtgagcgtgggtctcgcggtatcattgcagcactggggccagatggtaagccctcccgtatcgtagttatctacacgacggggagtcaggcaactatggatgaacgaaatagacagatcgctgagataggtgcctcactgattaagcattggtaactgtcagaccaagtttactcatatatactttagattgatttaaaacttcatttttaatttaaaaggatctaggtgaagatcctttttgataatctcatgaccaaaatcccttaacgtgagttttcgttccactgagcgtcagaccccgtagaaaagatcaaaggatcttcttgagatcctttttttctgcgcgtaatctgctgcttgcaaacaaaaaaaccaccgctaccagcggtggtttgtttgccggatcaagagctaccaactctttttccgaaggtaactggcttcagcagagcgcagataccaaatactgttcttctagtgtagccgtagttaggccaccacttcaagaactctgtagcaccgcctacatacctcgctctgctaatcctgttaccagtggctgctgccagtggcgataagtcgtgtcttaccgggttggactcaagacgatagttaccggataaggcgcagcggtcgggctgaacggggggttcgtgcacacagcccagcttggagcgaacgacctacaccgaactgagatacctacagcgtgagctatgagaaagcgccacgcttcccgaagggagaaaggcggacaggtatccggtaagcggcagggtcggaacaggagagcgcacgagggagcttccagggggaaacgcctggtatctttatagtcctgtcgggtttcgccacctctgacttgagcgtcgatttttgtgatgctcgtcaggggggcggagcctatggaaaaacgccagcaacgcggcctttttacggttcctggccttttgctggccttttgctcacatgttctttcctgcgttatcccctgattctgtggataaccgtattaccgcctttgag

SEQ ID NO: 169 - RNA, 19 nt, synthetic construct
  source 1..19: mol_type = other RNA
acaaagaggaagagagacg

SEQ ID NO: 170 - protein, 180 aa, synthetic construct
MYNAPRFFCRSAAVSDHEFNDEYWMRHALTLAKRAREEGEVPVGAVLVLNNQVIGEGWNRAIGLHDPTAHAEIMALRQGGLVLQNYRLIDATLYVTFEPCVMCAGAMVHSRISRLVFGVRNSKRGAAGSLINVLNYPGMNHRVEITEGILAESCSAMLCDFYRWPREVFNALKKARQEEG

SEQ ID NO: 171 - protein, 5 aa, synthetic construct
GGGGS

SEQ ID NO: 172 - protein, 4 aa, synthetic construct
SGGS

SEQ ID NO: 173 - protein, 24 aa, synthetic construct
SGGSSGSETPGTSESATPESSGGS

SEQ ID NO: 174 - protein, 32 aa, synthetic construct
SGGSSGGSSGSETPGTSESATPESSGGSSGGS

SEQ ID NO: 175 - protein, 104 aa, synthetic construct
GGSGGSPGSPAGSPTSTEEGTSESATPESGPGTSTEPSEGSAPGSPAGSPTSTEEGTSTEPSEGSAPGTSTEPSEGSAPGTSESATPESGPGSEPATSGGSGGS

SEQ ID NO: 176 - protein, 16 aa, synthetic construct
SGSETPGTSESATPES

SEQ ID NO: 177 - protein, 24 aa, synthetic construct
SGGSSGGSSGSETPGTSESATPES

SEQ ID NO: 178 - protein, 40 aa, synthetic construct
SGGSSGGSSGSETPGTSESATPESSGGSSGGSSGGSSGGS

SEQ ID NO: 179 - protein, 64 aa, synthetic construct
SGGSSGGSSGSETPGTSESATPESSGGSSGGSSGGSSGGSSGSETPGTSESATPESSGGSSGGS

SEQ ID NO: 180 - protein, 92 aa, synthetic construct
PGSPAGSPTSTEEGTSESATPESGPGTSTEPSEGSAPGSPAGSPTSTEEGTSTEPSEGSAPGTSTEPSEGSAPGTSESATPESGPGSEPATS

SEQ ID NO: 181 - protein, 18 aa, synthetic construct
KRTADGSEFESPKKKRKV

SEQ ID NO: 182 - protein, 16 aa, synthetic construct
KRPAATKKAGQAKKKK

SEQ ID NO: 183 - protein, 17 aa, synthetic construct
KKTELQTTNAENKTKKL

SEQ ID NO: 184 - protein, 19 aa, synthetic construct
KRGINDRNFWRGENGRKTR

SEQ ID NO: 185 - protein, 16 aa, synthetic construct
RKSGKIAAIVVKRPRK

SEQ ID NO: 186 - protein, 7 aa, synthetic construct
PKKKRKV

SEQ ID NO: 187 - protein, 28 aa, synthetic construct
MDSLLMNRRKFLYQFKNVRWAKGRRETY

SEQ ID NO: 188 - protein, 19 aa, synthetic construct
MKRTADGSEFESPKKKRKV

SEQ ID NO: 189 - protein, 21 aa, synthetic construct
SGGSKRTADGSEFEPKKKRKV

SEQ ID NO: 190 - protein, 1619 aa, synthetic construct
MKRTADGSEFESPKKKRKVMYNAPRFFCRSAAVSDHEFNDEYWMRHALTLAKRAREEGEVPVGAVLVLNNQVIGEGWNRAIGLHDPTAHAEIMALRQGGLVLQNYRLIDATLYVTFEPCVMCAGAMVHSRISRLVFGVRNSKRGAAGSLINVLNYPGMNHRVEITEGILAESCSAMLCDFYRWPREVFNALKKARQEEGSGGSSGGSSGSETPGTSESATPESSGGSSGGSDKKYSIGLAIGTNSVGWAVITDEYKVPSKKFKVLGNTDRHSIKKNLIGALLFDSGETAEATRLKRTARRRYTRRKNRICYLQEIFSNEMAKVDDSFFHRLEESFLVEEDKKHERHPIFGNIVDEVAYHEKYPTIYHLRKKLVDSTDKADLRLIYLALAHMIKFRGHFLIEGDLNPDNSDVDKLFIQLVQTYNQLFEENPINASGVDAKAILSARLSKSRRLENLIAQLPGEKKNGLFGNLIALSLGLTPNFKSNFDLAEDAKLQLSKDTYDDDLDNLLAQIGDQYADLFLAAKNLSDAILLSDILRVNTEITKAPLSASMIKRYDEHHQDLTLLKALVRQQLPEKYKEIFFDQSKNGYAGYIDGGASQEEFYKFIKPILEKMDGTEELLVKLNREDLLRKQRTFDNGSIPHQIHLGELHAILRRQEDFYPFLKDNREKIEKILTFRIPYYVGPLARGNSRFAWMTRKSEETITPWNFEEVVDKGASAQSFIERMTNFDKNLPNEKVLPKHSLLYEYFTVYNELTKVKYVTEGMRKPAFLSGEQKKAIVDLLFKTNRKVTVKQLKEDYFKKIECFDSVEISGVEDRFNASLGTYHDLLKIIKDKDFLDNEENEDILEDIVLTLTLFEDREMIEERLKTYAHLFDDKVMKQLKRRRYTGWGRLSRKLINGIRDKQSGKTILDFLKSDGFANRNFMQLIHDDSLTFKEDIQKAQVSGQGDSLHEHIANLAGSPAIKKGILQTVKVVDELVKVMGRHKPENIVIEMARENQTTQKGQKNSRERMKRIEEGIKELGSQILKEHPVENTQLQNEKLYLYYLQNGRDMYVDQELDINRLSDYDVDHIVPQSFLKDDSIDNKVLTRSDKNRGKSDNVPSEEVVKKMKNYWRQLLNAKLITQRKFDNLTKAERGGLSELDKAGFIKRQLVETRQITKHVAQILDSRMNTKYDENDKLIREVKVITLKSKLVSDFRKDFQFYKVREINNYHHAHDAYLNAVVGTALIKKYPKLESEFVYGDYKVYDVRKMIAKSEQEIGKATAKYFFYSNIMNFFKTEITLANGEIRKRPLIETNGETGEIVWDKGRDFATVRKVLSMPQVNIVKKTEVQTGGFSKESILPKRNSDKLIARKKDWDPKKYGGFDSPTVAYSVLVVAKVEKGKSKKLKSVKELLGITIMERSSFEKNPIDFLEAKGYKEVKKDLIIKLPKYSLFELENGRKRMLASAGELQKGNELALPSKYVNFLYLASHYEKLKGSPEDNEQKQLFVEQHKHYLDEIIEQISEFSKRVILADANLDKVLSAYNKHRDKPIREQAENIIHLFTLTNLGAPAAFKYFDTTIDRKRYTSTKEVLDATLIHQSITGLYETRIDLSQLGGDSGGSKRTADGSEFEPKKKRKV

SEQ ID NO: 191 - protein, 1619 aa, synthetic construct
MKRTADGSEFESPKKKRKVMYNAPRFFCRSAAVTEKEYQDEYWMRHALTLAKRAREEGEVPVGAVLVLNNQVIGEGWNRAIGLHDPTAHAEIMALRQGGLVLQNYRLIDATLYVTFEPCVMCAGAMVHSRISRLVFGVRNSKRGAAGSLINVLNYPGMNHRVEITEGILAESCSAMLCDFYRWPREVFNALKKARQEEGSGGSSGGSSGSETPGTSESATPESSGGSSGGSDKKYSIGLAIGTNSVGWAVITDEYKVPSKKFKVLGNTDRHSIKKNLIGALLFDSGETAEATRLKRTARRRYTRRKNRICYLQEIFSNEMAKVDDSFFHRLEESFLVEEDKKHERHPIFGNIVDEVAYHEKYPTIYHLRKKLVDSTDKADLRLIYLALAHMIKFRGHFLIEGDLNPDNSDVDKLFIQLVQTYNQLFEENPINASGVDAKAILSARLSKSRRLENLIAQLPGEKKNGLFGNLIALSLGLTPNFKSNFDLAEDAKLQLSKDTYDDDLDNLLAQIGDQYADLFLAAKNLSDAILLSDILRVNTEITKAPLSASMIKRYDEHHQDLTLLKALVRQQLPEKYKEIFFDQSKNGYAGYIDGGASQEEFYKFIKPILEKMDGTEELLVKLNREDLLRKQRTFDNGSIPHQIHLGELHAILRRQEDFYPFLKDNREKIEKILTFRIPYYVGPLARGNSRFAWMTRKSEETITPWNFEEVVDKGASAQSFIERMTNFDKNLPNEKVLPKHSLLYEYFTVYNELTKVKYVTEGMRKPAFLSGEQKKAIVDLLFKTNRKVTVKQLKEDYFKKIECFDSVEISGVEDRFNASLGTYHDLLKIIKDKDFLDNEENEDILEDIVLTLTLFEDREMIEERLKTYAHLFDDKVMKQLKRRRYTGWGRLSRKLINGIRDKQSGKTILDFLKSDGFANRNFMQLIHDDSLTFKEDIQKAQVSGQGDSLHEHIANLAGSPAIKKGILQTVKVVDELVKVMGRHKPENIVIEMARENQTTQKGQKNSRERMKRIEEGIKELGSQILKEHPVENTQLQNEKLYLYYLQNGRDMYVDQELDINRLSDYDVDHIVPQSFLKDDSIDNKVLTRSDKNRGKSDNVPSEEVVKKMKNYWRQLLNAKLITQRKFDNLTKAERGGLSELDKAGFIKRQLVETRQITKHVAQILDSRMNTKYDENDKLIREVKVITLKSKLVSDFRKDFQFYKVREINNYHHAHDAYLNAVVGTALIKKYPKLESEFVYGDYKVYDVRKMIAKSEQEIGKATAKYFFYSNIMNFFKTEITLANGEIRKRPLIETNGETGEIVWDKGRDFATVRKVLSMPQVNIVKKTEVQTGGFSKESILPKRNSDKLIARKKDWDPKKYGGFDSPTVAYSVLVVAKVEKGKSKKLKSVKELLGITIMERSSFEKNPIDFLEAKGYKEVKKDLIIKLPKYSLFELENGRKRMLASAGELQKGNELALPSKYVNFLYLASHYEKLKGSPEDNEQKQLFVEQHKHYLDEIIEQISEFSKRVILADANLDKVLSAYNKHRDKPIREQAENIIHLFTLTNLGAPAAFKYFDTTIDRKRYTSTKEVLDATLIHQSITGLYETRIDLSQLGGDSGGSKRTADGSEFEPKKKRKV

SEQ ID NO: 192 - protein, 1619 aa, synthetic construct
MKRTADGSEFESPKKKRKVMYNAPRFFCRSAAVSDHEFNDDFFMKRAITLAKRAREEGEVPVGAVLVLNNQVIGEGWNRAIGLHDPTAHAEIMALRQGGLVLQNYRLIDATLYVTFEPCVMCAGAMVHSRISRLVFGVRNSKRGAAGSLINVLNYPGMNHRVEITEGILAESCSAMLCDFYRWPREVFNALKKARQEEGSGGSSGGSSGSETPGTSESATPESSGGSSGGSDKKYSIGLAIGTNSVGWAVITDEYKVPSKKFKVLGNTDRHSIKKNLIGALLFDSGETAEATRLKRTARRRYTRRKNRICYLQEIFSNEMAKVDDSFFHRLEESFLVEEDKKHERHPIFGNIVDEVAYHEKYPTIYHLRKKLVDSTDKADLRLIYLALAHMIKFRGHFLIEGDLNPDNSDVDKLFIQLVQTYNQLFEENPINASGVDAKAILSARLSKSRRLENLIAQLPGEKKNGLFGNLIALSLGLTPNFKSNFDLAEDAKLQLSKDTYDDDLDNLLAQIGDQYADLFLAAKNLSDAILLSDILRVNTEITKAPLSASMIKRYDEHHQDLTLLKALVRQQLPEKYKEIFFDQSKNGYAGYIDGGASQEEFYKFIKPILEKMDGTEELLVKLNREDLLRKQRTFDNGSIPHQIHLGELHAILRRQEDFYPFLKDNREKIEKILTFRIPYYVGPLARGNSRFAWMTRKSEETITPWNFEEVVDKGASAQSFIERMTNFDKNLPNEKVLPKHSLLYEYFTVYNELTKVKYVTEGMRKPAFLSGEQKKAIVDLLFKTNRKVTVKQLKEDYFKKIECFDSVEISGVEDRFNASLGTYHDLLKIIKDKDFLDNEENEDILEDIVLTLTLFEDREMIEERLKTYAHLFDDKVMKQLKRRRYTGWGRLSRKLINGIRDKQSGKTILDFLKSDGFANRNFMQLIHDDSLTFKEDIQKAQVSGQGDSLHEHIANLAGSPAIKKGILQTVKVVDELVKVMGRHKPENIVIEMARENQTTQKGQKNSRERMKRIEEGIKELGSQILKEHPVENTQLQNEKLYLYYLQNGRDMYVDQELDINRLSDYDVDHIVPQSFLKDDSIDNKVLTRSDKNRGKSDNVPSEEVVKKMKNYWRQLLNAKLITQRKFDNLTKAERGGLSELDKAGFIKRQLVETRQITKHVAQILDSRMNTKYDENDKLIREVKVITLKSKLVSDFRKDFQFYKVREINNYHHAHDAYLNAVVGTALIKKYPKLESEFVYGDYKVYDVRKMIAKSEQEIGKATAKYFFYSNIMNFFKTEITLANGEIRKRPLIETNGETGEIVWDKGRDFATVRKVLSMPQVNIVKKTEVQTGGFSKESILPKRNSDKLIARKKDWDPKKYGGFDSPTVAYSVLVVAKVEKGKSKKLKSVKELLGITIMERSSFEKNPIDFLEAKGYKEVKKDLIIKLPKYSLFELENGRKRMLASAGELQKGNELALPSKYVNFLYLASHYEKLKGSPEDNEQKQLFVEQHKHYLDEIIEQISEFSKRVILADANLDKVLSAYNKHRDKPIREQAENIIHLFTLTNLGAPAAFKYFDTTIDRKRYTSTKEVLDATLIHQSITGLYETRIDLSQLGGDSGGSKRTADGSEFEPKKKRKV

SEQ ID NO: 193 - protein, 1619 aa, synthetic construct
MKRTADGSEFESPKKKRKVMYNAPRFFCRSAAVSDHEFNDEYWMRHALTLARKSREEGEVPVGAVLVLNNQVIGEGWNRAIGLHDPTAHAEIMALRQGGLVLQNYRLIDATLYVTFEPCVMCAGAMVHSRISRLVFGVRNSKRGAAGSLINVLNYPGMNHRVEITEGILAESCSAMLCDFYRWPREVFNALKKARQEEGSGGSSGGSSGSETPGTSESATPESSGGSSGGSDKKYSIGLAIGTNSVGWAVITDEYKVPSKKFKVLGNTDRHSIKKNLIGALLFDSGETAEATRLKRTARRRYTRRKNRICYLQEIFSNEMAKVDDSFFHRLEESFLVEEDKKHERHPIFGNIVDEVAYHEKYPTIYHLRKKLVDSTDKADLRLIYLALAHMIKFRGHFLIEGDLNPDNSDVDKLFIQLVQTYNQLFEENPINASGVDAKAILSARLSKSRRLENLIAQLPGEKKNGLFGNLIALSLGLTPNFKSNFDLAEDAKLQLSKDTYDDDLDNLLAQIGDQYADLFLAAKNLSDAILLSDILRVNTEITKAPLSASMIKRYDEHHQDLTLLKALVRQQLPEKYKEIFFDQSKNGYAGYIDGGASQEEFYKFIKPILEKMDGTEELLVKLNREDLLRKQRTFDNGSIPHQIHLGELHAILRRQEDFYPFLKDNREKIEKILTFRIPYYVGPLARGNSRFAWMTRKSEETITPWNFEEVVDKGASAQSFIERMTNFDKNLPNEKVLPKHSLLYEYFTVYNELTKVKYVTEGMRKPAFLSGEQKKAIVDLLFKTNRKVTVKQLKEDYFKKIECFDSVEISGVEDRFNASLGTYHDLLKIIKDKDFLDNEENEDILEDIVLTLTLFEDREMIEERLKTYAHLFDDKVMKQLKRRRYTGWGRLSRKLINGIRDKQSGKTILDFLKSDGFANRNFMQLIHDDSLTFKEDIQKAQVSGQGDSLHEHIANLAGSPAIKKGILQTVKVVDELVKVMGRHKPENIVIEMARENQTTQKGQKNSRERMKRIEEGIKELGSQILKEHPVENTQLQNEKLYLYYLQNGRDMYVDQELDINRLSDYDVDHIVPQSFLKDDSIDNKVLTRSDKNRGKSDNVPSEEVVKKMKNYWRQLLNAKLITQRKFDNLTKAERGGLSELDKAGFIKRQLVETRQITKHVAQILDSRMNTKYDENDKLIREVKVITLKSKLVSDFRKDFQFYKVREINNYHHAHDAYLNAVVGTALIKKYPKLESEFVYGDYKVYDVRKMIAKSEQEIGKATAKYFFYSNIMNFFKTEITLANGEIRKRPLIETNGETGEIVWDKGRDFATVRKVLSMPQVNIVKKTEVQTGGFSKESILPKRNSDKLIARKKDWDPKKYGGFDSPTVAYSVLVVAKVEKGKSKKLKSVKELLGITIMERSSFEKNPIDFLEAKGYKEVKKDLIIKLPKYSLFELENGRKRMLASAGELQKGNELALPSKYVNFLYLASHYEKLKGSPEDNEQKQLFVEQHKHYLDEIIEQISEFSKRVILADANLDKVLSAYNKHRDKPIREQAENIIHLFTLTNLGAPAAFKYFDTTIDRKRYTSTKEVLDATLIHQSITGLYETRIDLSQLGGDSGGSKRTADGSEFEPKKKRKV

SEQ ID NO: 194 - protein, 1619 aa, synthetic construct
MKRTADGSEFESPKKKRKVMYNAPRFFCRSAAVSDHEFNDEYWMRHALTLAKRAREEGEVPVGAVLVLNNQVIGEGWNRAIGLHDPTAHAEIMALRQGANAINSWRLIDATLYVTFEPCVMCAGAMVHSRISRLVFGVRNSKRGAAGSLINVLNYPGMNHRVEITEGILAESCSAMLCDFYRWPREVFNALKKARQEEGSGGSSGGSSGSETPGTSESATPESSGGSSGGSDKKYSIGLAIGTNSVGWAVITDEYKVPSKKFKVLGNTDRHSIKKNLIGALLFDSGETAEATRLKRTARRRYTRRKNRICYLQEIFSNEMAKVDDSFFHRLEESFLVEEDKKHERHPIFGNIVDEVAYHEKYPTIYHLRKKLVDSTDKADLRLIYLALAHMIKFRGHFLIEGDLNPDNSDVDKLFIQLVQTYNQLFEENPINASGVDAKAILSARLSKSRRLENLIAQLPGEKKNGLFGNLIALSLGLTPNFKSNFDLAEDAKLQLSKDTYDDDLDNLLAQIGDQYADLFLAAKNLSDAILLSDILRVNTEITKAPLSASMIKRYDEHHQDLTLLKALVRQQLPEKYKEIFFDQSKNGYAGYIDGGASQEEFYKFIKPILEKMDGTEELLVKLNREDLLRKQRTFDNGSIPHQIHLGELHAILRRQEDFYPFLKDNREKIEKILTFRIPYYVGPLARGNSRFAWMTRKSEETITPWNFEEVVDKGASAQSFIERMTNFDKNLPNEKVLPKHSLLYEYFTVYNELTKVKYVTEGMRKPAFLSGEQKKAIVDLLFKTNRKVTVKQLKEDYFKKIECFDSVEISGVEDRFNASLGTYHDLLKIIKDKDFLDNEENEDILEDIVLTLTLFEDREMIEERLKTYAHLFDDKVMKQLKRRRYTGWGRLSRKLINGIRDKQSGKTILDFLKSDGFANRNFMQLIHDDSLTFKEDIQKAQVSGQGDSLHEHIANLAGSPAIKKGILQTVKVVDELVKVMGRHKPENIVIEMARENQTTQKGQKNSRERMKRIEEGIKELGSQILKEHPVENTQLQNEKLYLYYLQNGRDMYVDQELDINRLSDYDVDHIVPQSFLKDDSIDNKVLTRSDKNRGKSDNVPSEEVVKKMKNYWRQLLNAKLITQRKFDNLTKAERGGLSELDKAGFIKRQLVETRQITKHVAQILDSRMNTKYDENDKLIREVKVITLKSKLVSDFRKDFQFYKVREINNYHHAHDAYLNAVVGTALIKKYPKLESEFVYGDYKVYDVRKMIAKSEQEIGKATAKYFFYSNIMNFFKTEITLANGEIRKRPLIETNGETGEIVWDKGRDFATVRKVLSMPQVNIVKKTEVQTGGFSKESILPKRNSDKLIARKKDWDPKKYGGFDSPTVAYSVLVVAKVEKGKSKKLKSVKELLGITIMERSSFEKNPIDFLEAKGYKEVKKDLIIKLPKYSLFELENGRKRMLASAGELQKGNELALPSKYVNFLYLASHYEKLKGSPEDNEQKQLFVEQHKHYLDEIIEQISEFSKRVILADANLDKVLSAYNKHRDKPIREQAENIIHLFTLTNLGAPAAFKYFDTTIDRKRYTSTKEVLDATLIHQSITGLYETRIDLSQLGGDSGGSKRTADGSEFEPKKKRKV

SEQ ID NO: 195 - protein, 1619 aa, synthetic construct
MKRTADGSEFESPKKKRKVMYNAPRFFCRSAAVSDHEFNDEYWMRHALTLAKRAREEGEVPVGAVLVLNNQVIGEGWNRAIGLHDPTAHAEIMALRQGGLVLQNYRLLGTDLYVTFEPCVMCAGAMVHSRISRLVFGVRNSKRGAAGSLINVLNYPGMNHRVEITEGILAESCSAMLCDFYRWPREVFNALKKARQEEGSGGSSGGSSGSETPGTSESATPESSGGSSGGSDKKYSIGLAIGTNSVGWAVITDEYKVPSKKFKVLGNTDRHSIKKNLIGALLFDSGETAEATRLKRTARRRYTRRKNRICYLQEIFSNEMAKVDDSFFHRLEESFLVEEDKKHERHPIFGNIVDEVAYHEKYPTIYHLRKKLVDSTDKADLRLIYLALAHMIKFRGHFLIEGDLNPDNSDVDKLFIQLVQTYNQLFEENPINASGVDAKAILSARLSKSRRLENLIAQLPGEKKNGLFGNLIALSLGLTPNFKSNFDLAEDAKLQLSKDTYDDDLDNLLAQIGDQYADLFLAAKNLSDAILLSDILRVNTEITKAPLSASMIKRYDEHHQDLTLLKALVRQQLPEKYKEIFFDQSKNGYAGYIDGGASQEEFYKFIKPILEKMDGTEELLVKLNREDLLRKQRTFDNGSIPHQIHLGELHAILRRQEDFYPFLKDNREKIEKILTFRIPYYVGPLARGNSRFAWMTRKSEETITPWNFEEVVDKGASAQSFIERMTNFDKNLPNEKVLPKHSLLYEYFTVYNELTKVKYVTEGMRKPAFLSGEQKKAIVDLLFKTNRKVTVKQLKEDYFKKIECFDSVEISGVEDRFNASLGTYHDLLKIIKDKDFLDNEENEDILEDIVLTLTLFEDREMIEERLKTYAHLFDDKVMKQLKRRRYTGWGRLSRKLINGIRDKQSGKTILDFLKSDGFANRNFMQLIHDDSLTFKEDIQKAQVSGQGDSLHEHIANLAGSPAIKKGILQTVKVVDELVKVMGRHKPENIVIEMARENQTTQKGQKNSRERMKRIEEGIKELGSQILKEHPVENTQLQNEKLYLYYLQNGRDMYVDQELDINRLSDYDVDHIVPQSFLKDDSIDNKVLTRSDKNRGKSDNVPSEEVVKKMKNYWRQLLNAKLITQRKFDNLTKAERGGLSELDKAGFIKRQLVETRQITKHVAQILDSRMNTKYDENDKLIREVKVITLKSKLVSDFRKDFQFYKVREINNYHHAHDAYLNAVVGTALIKKYPKLESEFVYGDYKVYDVRKMIAKSEQEIGKATAKYFFYSNIMNFFKTEITLANGEIRKRPLIETNGETGEIVWDKGRDFATVRKVLSMPQVNIVKKTEVQTGGFSKESILPKRNSDKLIARKKDWDPKKYGGFDSPTVAYSVLVVAKVEKGKSKKLKSVKELLGITIMERSSFEKNPIDFLEAKGYKEVKKDLIIKLPKYSLFELENGRKRMLASAGELQKGNELALPSKYVNFLYLASHYEKLKGSPEDNEQKQLFVEQHKHYLDEIIEQISEFSKRVILADANLDKVLSAYNKHRDKPIREQAENIIHLFTLTNLGAPAAFKYFDTTIDRKRYTSTKEVLDATLIHQSITGLYETRIDLSQLGGDSGGSKRTADGSEFEPKKKRKV

SEQ ID NO: 196 - protein, 1619 aa, synthetic construct
MKRTADGSEFESPKKKRKVMYNAPRFFCRSAAVSDHEFNDEYWMRHALTLAKRAREEGEVPVGAVLVLNNQVIGEGWNRAIGLHDPTAHAEIMALRQGGLVLQNYRLIDATLYVTFEPCVMCAGAMVHSRLKKLVFGVRNSKRGAAGSLINVLNYPGMNHRVEITEGILAESCSAMLCDFYRWPREVFNALKKARQEEGSGGSSGGSSGSETPGTSESATPESSGGSSGGSDKKYSIGLAIGTNSVGWAVITDEYKVPSKKFKVLGNTDRHSIKKNLIGALLFDSGETAEATRLKRTARRRYTRRKNRICYLQEIFSNEMAKVDDSFFHRLEESFLVEEDKKHERHPIFGNIVDEVAYHEKYPTIYHLRKKLVDSTDKADLRLIYLALAHMIKFRGHFLIEGDLNPDNSDVDKLFIQLVQTYNQLFEENPINASGVDAKAILSARLSKSRRLENLIAQLPGEKKNGLFGNLIALSLGLTPNFKSNFDLAEDAKLQLSKDTYDDDLDNLLAQIGDQYADLFLAAKNLSDAILLSDILRVNTEITKAPLSASMIKRYDEHHQDLTLLKALVRQQLPEKYKEIFFDQSKNGYAGYIDGGASQEEFYKFIKPILEKMDGTEELLVKLNREDLLRKQRTFDNGSIPHQIHLGELHAILRRQEDFYPFLKDNREKIEKILTFRIPYYVGPLARGNSRFAWMTRKSEETITPWNFEEVVDKGASAQSFIERMTNFDKNLPNEKVLPKHSLLYEYFTVYNELTKVKYVTEGMRKPAFLSGEQKKAIVDLLFKTNRKVTVKQLKEDYFKKIECFDSVEISGVEDRFNASLGTYHDLLKIIKDKDFLDNEENEDILEDIVLTLTLFEDREMIEERLKTYAHLFDDKVMKQLKRRRYTGWGRLSRKLINGIRDKQSGKTILDFLKSDGFANRNFMQLIHDDSLTFKEDIQKAQVSGQGDSLHEHIANLAGSPAIKKGILQTVKVVDELVKVMGRHKPENIVIEMARENQTTQKGQKNSRERMKRIEEGIKELGSQILKEHPVENTQLQNEKLYLYYLQNGRDMYVDQELDINRLSDYDVDHIVPQSFLKDDSIDNKVLTRSDKNRGKSDNVPSEEVVKKMKNYWRQLLNAKLITQRKFDNLTKAERGGLSELDKAGFIKRQLVETRQITKHVAQILDSRMNTKYDENDKLIREVKVITLKSKLVSDFRKDFQFYKVREINNYHHAHDAYLNAVVGTALIKKYPKLESEFVYGDYKVYDVRKMIAKSEQEIGKATAKYFFYSNIMNFFKTEITLANGEIRKRPLIETNGETGEIVWDKGRDFATVRKVLSMPQVNIVKKTEVQTGGFSKESILPKRNSDKLIARKKDWDPKKYGGFDSPTVAYSVLVVAKVEKGKSKKLKSVKELLGITIMERSSFEKNPIDFLEAKGYKEVKKDLIIKLPKYSLFELENGRKRMLASAGELQKGNELALPSKYVNFLYLASHYEKLKGSPEDNEQKQLFVEQHKHYLDEIIEQISEFSKRVILADANLDKVLSAYNKHRDKPIREQAENIIHLFTLTNLGAPAAFKYFDTTIDRKRYTSTKEVLDATLIHQSITGLYETRIDLSQLGGDSGGSKRTADGSEFEPKKKRKV

SEQ ID NO: 197 - protein, 1619 aa, synthetic construct
MKRTADGSEFESPKKKRKVMYNAPRFFCRSAAVSDHEFNDEYWMRHALTLAKRAREEGEVPVGAVLVLNNQVIGEGWNRAIGLHDPTAHAEIMALRQGGLVLQNYRLIDATLYVTFEPCVMCAGAMVHSRISRLVFGVRNSKRGAAGSLIKIFHYPGMNHRVEITEGILAESCSAMLCDFYRWPREVFNALKKARQEEGSGGSSGGSSGSETPGTSESATPESSGGSSGGSDKKYSIGLAIGTNSVGWAVITDEYKVPSKKFKVLGNTDRHSIKKNLIGALLFDSGETAEATRLKRTARRRYTRRKNRICYLQEIFSNEMAKVDDSFFHRLEESFLVEEDKKHERHPIFGNIVDEVAYHEKYPTIYHLRKKLVDSTDKADLRLIYLALAHMIKFRGHFLIEGDLNPDNSDVDKLFIQLVQTYNQLFEENPINASGVDAKAILSARLSKSRRLENLIAQLPGEKKNGLFGNLIALSLGLTPNFKSNFDLAEDAKLQLSKDTYDDDLDNLLAQIGDQYADLFLAAKNLSDAILLSDILRVNTEITKAPLSASMIKRYDEHHQDLTLLKALVRQQLPEKYKEIFFDQSKNGYAGYIDGGASQEEFYKFIKPILEKMDGTEELLVKLNREDLLRKQRTFDNGSIPHQIHLGELHAILRRQEDFYPFLKDNREKIEKILTFRIPYYVGPLARGNSRFAWMTRKSEETITPWNFEEVVDKGASAQSFIERMTNFDKNLPNEKVLPKHSLLYEYFTVYNELTKVKYVTEGMRKPAFLSGEQKKAIVDLLFKTNRKVTVKQLKEDYFKKIECFDSVEISGVEDRFNASLGTYHDLLKIIKDKDFLDNEENEDILEDIVLTLTLFEDREMIEERLKTYAHLFDDKVMKQLKRRRYTGWGRLSRKLINGIRDKQSGKTILDFLKSDGFANRNFMQLIHDDSLTFKEDIQKAQVSGQGDSLHEHIANLAGSPAIKKGILQTVKVVDELVKVMGRHKPENIVIEMARENQTTQKGQKNSRERMKRIEEGIKELGSQILKEHPVENTQLQNEKLYLYYLQNGRDMYVDQELDINRLSDYDVDHIVPQSFLKDDSIDNKVLTRSDKNRGKSDNVPSEEVVKKMKNYWRQLLNAKLITQRKFDNLTKAERGGLSELDKAGFIKRQLVETRQITKHVAQILDSRMNTKYDENDKLIREVKVITLKSKLVSDFRKDFQFYKVREINNYHHAHDAYLNAVVGTALIKKYPKLESEFVYGDYKVYDVRKMIAKSEQEIGKATAKYFFYSNIMNFFKTEITLANGEIRKRPLIETNGETGEIVWDKGRDFATVRKVLSMPQVNIVKKTEVQTGGFSKESILPKRNSDKLIARKKDWDPKKYGGFDSPTVAYSVLVVAKVEKGKSKKLKSVKELLGITIMERSSFEKNPIDFLEAKGYKEVKKDLIIKLPKYSLFELENGRKRMLASAGELQKGNELALPSKYVNFLYLASHYEKLKGSPEDNEQKQLFVEQHKHYLDEIIEQISEFSKRVILADANLDKVLSAYNKHRDKPIREQAENIIHLFTLTNLGAPAAFKYFDTTIDRKRYTSTKEVLDATLIHQSITGLYETRIDLSQLGGDSGGSKRTADGSEFEPKKKRKV

SEQ ID NO: 198 - protein, 1619 aa, synthetic construct
MKRTADGSEFESPKKKRKVMYNAPRFFCRSAAVSDHEFNDEYWMRHALTLAKRAREEGEVPVGAVLVLNNQVIGEGWNRAIGLHDPTAHAEIMALRQGGLVLQNYRLIDATLYVTFEPCVMCAGAMVHSRISRLVFGVRNSKRGAAGSLINVLNYFALNHRVEITEGILAESCSAMLCDFYRWPREVFNALKKARQEEGSGGSSGGSSGSETPGTSESATPESSGGSSGGSDKKYSIGLAIGTNSVGWAVITDEYKVPSKKFKVLGNTDRHSIKKNLIGALLFDSGETAEATRLKRTARRRYTRRKNRICYLQEIFSNEMAKVDDSFFHRLEESFLVEEDKKHERHPIFGNIVDEVAYHEKYPTIYHLRKKLVDSTDKADLRLIYLALAHMIKFRGHFLIEGDLNPDNSDVDKLFIQLVQTYNQLFEENPINASGVDAKAILSARLSKSRRLENLIAQLPGEKKNGLFGNLIALSLGLTPNFKSNFDLAEDAKLQLSKDTYDDDLDNLLAQIGDQYADLFLAAKNLSDAILLSDILRVNTEITKAPLSASMIKRYDEHHQDLTLLKALVRQQLPEKYKEIFFDQSKNGYAGYIDGGASQEEFYKFIKPILEKMDGTEELLVKLNREDLLRKQRTFDNGSIPHQIHLGELHAILRRQEDFYPFLKDNREKIEKILTFRIPYYVGPLARGNSRFAWMTRKSEETITPWNFEEVVDKGASAQSFIERMTNFDKNLPNEKVLPKHSLLYEYFTVYNELTKVKYVTEGMRKPAFLSGEQKKAIVDLLFKTNRKVTVKQLKEDYFKKIECFDSVEISGVEDRFNASLGTYHDLLKIIKDKDFLDNEENEDILEDIVLTLTLFEDREMIEERLKTYAHLFDDKVMKQLKRRRYTGWGRLSRKLINGIRDKQSGKTILDFLKSDGFANRNFMQLIHDDSLTFKEDIQKAQVSGQGDSLHEHIANLAGSPAIKKGILQTVKVVDELVKVMGRHKPENIVIEMARENQTTQKGQKNSRERMKRIEEGIKELGSQILKEHPVENTQLQNEKLYLYYLQNGRDMYVDQELDINRLSDYDVDHIVPQSFLKDDSIDNKVLTRSDKNRGKSDNVPSEEVVKKMKNYWRQLLNAKLITQRKFDNLTKAERGGLSELDKAGFIKRQLVETRQITKHVAQILDSRMNTKYDENDKLIREVKVITLKSKLVSDFRKDFQFYKVREINNYHHAHDAYLNAVVGTALIKKYPKLESEFVYGDYKVYDVRKMIAKSEQEIGKATAKYFFYSNIMNFFKTEITLANGEIRKRPLIETNGETGEIVWDKGRDFATVRKVLSMPQVNIVKKTEVQTGGFSKESILPKRNSDKLIARKKDWDPKKYGGFDSPTVAYSVLVVAKVEKGKSKKLKSVKELLGITIMERSSFEKNPIDFLEAKGYKEVKKDLIIKLPKYSLFELENGRKRMLASAGELQKGNELALPSKYVNFLYLASHYEKLKGSPEDNEQKQLFVEQHKHYLDEIIEQISEFSKRVILADANLDKVLSAYNKHRDKPIREQAENIIHLFTLTNLGAPAAFKYFDTTIDRKRYTSTKEVLDATLIHQSITGLYETRIDLSQLGGDSGGSKRTADGSEFEPKKKRKV

SEQ ID NO: 199 - RNA, 76 nt, synthetic construct
  source 1..76: mol_type = other RNA
gttttagagctagaaatagcaagttaaaataaggctagtccgttatcaacttgaaaaagtggcaccgagtcggtgc

SEQ ID NO: 200 - protein, 1605 aa, synthetic construct
MKRTADGSEFESPKKKRKVSEVEFSHEYWMRHALTLAKRARDEREVPVGAVLVLNNRVIGEGWNRAIGLHDPTAHAEIMALRQGGLVMQNYRLIDATLYVTFEPCVMCAGAMIHSRIGRVVFGVRNSKRGAAGSLMNVLNYPGMNHRVEITEGILADECAALLCDFYRMPRQVFNAQKKAQSSINSGGSSGGSSGSETPGTSESATPESSGGSSGGSDKKYSIGLAIGTNSVGWAVITDEYKVPSKKFKVLGNTDRHSIKKNLIGALLFDSGETAEATRLKRTARRRYTRRKNRICYLQEIFSNEMAKVDDSFFHRLEESFLVEEDKKHERHPIFGNIVDEVAYHEKYPTIYHLRKKLVDSTDKADLRLIYLALAHMIKFRGHFLIEGDLNPDNSDVDKLFIQLVQTYNQLFEENPINASGVDAKAILSARLSKSRRLENLIAQLPGEKKNGLFGNLIALSLGLTPNFKSNFDLAEDAKLQLSKDTYDDDLDNLLAQIGDQYADLFLAAKNLSDAILLSDILRVNTEITKAPLSASMIKRYDEHHQDLTLLKALVRQQLPEKYKEIFFDQSKNGYAGYIDGGASQEEFYKFIKPILEKMDGTEELLVKLNREDLLRKQRTFDNGSIPHQIHLGELHAILRRQEDFYPFLKDNREKIEKILTFRIPYYVGPLARGNSRFAWMTRKSEETITPWNFEEVVDKGASAQSFIERMTNFDKNLPNEKVLPKHSLLYEYFTVYNELTKVKYVTEGMRKPAFLSGEQKKAIVDLLFKTNRKVTVKQLKEDYFKKIECFDSVEISGVEDRFNASLGTYHDLLKIIKDKDFLDNEENEDILEDIVLTLTLFEDREMIEERLKTYAHLFDDKVMKQLKRRRYTGWGRLSRKLINGIRDKQSGKTILDFLKSDGFANRNFMQLIHDDSLTFKEDIQKAQVSGQGDSLHEHIANLAGSPAIKKGILQTVKVVDELVKVMGRHKPENIVIEMARENQTTQKGQKNSRERMKRIEEGIKELGSQILKEHPVENTQLQNEKLYLYYLQNGRDMYVDQELDINRLSDYDVDHIVPQSFLKDDSIDNKVLTRSDKNRGKSDNVPSEEVVKKMKNYWRQLLNAKLITQRKFDNLTKAERGGLSELDKAGFIKRQLVETRQITKHVAQILDSRMNTKYDENDKLIREVKVITLKSKLVSDFRKDFQFYKVREINNYHHAHDAYLNAVVGTALIKKYPKLESEFVYGDYKVYDVRKMIAKSEQEIGKATAKYFFYSNIMNFFKTEITLANGEIRKRPLIETNGETGEIVWDKGRDFATVRKVLSMPQVNIVKKTEVQTGGFSKESILPKRNSDKLIARKKDWDPKKYGGFDSPTVAYSVLVVAKVEKGKSKKLKSVKELLGITIMERSSFEKNPIDFLEAKGYKEVKKDLIIKLPKYSLFELENGRKRMLASAGELQKGNELALPSKYVNFLYLASHYEKLKGSPEDNEQKQLFVEQHKHYLDEIIEQISEFSKRVILADANLDKVLSAYNKHRDKPIREQAENIIHLFTLTNLGAPAAFKYFDTTIDRKRYTSTKEVLDATLIHQSITGLYETRIDLSQLGGDSGGSKRTADGSEFEPKKKRKV

SEQ ID NO: 201 - DNA, 4818 bp, synthetic construct
  source 1..4818: mol_type = other DNA
atgaaacggacagccgacggaagcgagttcgagtcaccaaagaagaagcggaaagtctctgaggtggagttttcccacgagtactggatgagacatgccctgaccctggccaagagggcacgggatgagagggaggtgcctgtgggagccgtgctggtgctgaacaatagagtgatcggcgagggctggaacagagccatcggcctgcacgacccaacagcccatgccgaaattatggccctgagacagggcggcctggtcatgcagaactacagactgattgacgccaccctgtacgtgacattcgagccttgcgtgatgtgcgccggcgccatgatccactctaggatcggccgcgtggtgtttggcgtgaggaactcaaaaagaggcgccgcaggctccctgatgaacgtgctgaactaccccggcatgaatcaccgcgtcgaaattaccgagggaatcctggcagatgaatgtgccgccctgctgtgcgatttctatcggatgcctagacaggtgttcaatgctcagaagaaggcccagagctccatcaactccggaggatctagcggaggctcctctggctctgagacacctggcacaagcgagagcgcaacacctgaaagcagcgggggcagcagcggggggtcagacaagaagtacagcatcggcctggccatcggcaccaactctgtgggctgggccgtgatcaccgacgagtacaaggtgcccagcaagaaattcaaggtgctgggcaacaccgaccggcacagcatcaagaagaacctgatcggagccctgctgttcgacagcggcgaaacagccgaggccacccggctgaagagaaccgccagaagaagatacaccagacggaagaaccggatctgctatctgcaagagatcttcagcaacgagatggccaaggtggacgacagcttcttccacagactggaagagtccttcctggtggaagaggataagaagcacgagcggcaccccatcttcggcaacatcgtggacgaggtggcctaccacgagaagtaccccaccatctaccacctgagaaagaaactggtggacagcaccgacaaggccgacctgcggctgatctatctggccctggcccacatgatcaagttccggggccacttcctgatcgagggcgacctgaaccccgacaacagcgacgtggacaagctgttcatccagctggtgcagacctacaaccagctgttcgaggaaaaccccatcaacgccagcggcgtggacgccaaggccatcctgtctgccagactgagcaagagcagacggctggaaaatctgatcgcccagctgcccggcgagaagaagaatggcctgttcggaaacctgattgccctgagcctgggcctgacccccaacttcaagagcaacttcgacctggccgaggatgccaaactgcagctgagcaaggacacctacgacgacgacctggacaacctgctggcccagatcggcgaccagtacgccgacctgtttctggccgccaagaacctgtccgacgccatcctgctgagcgacatcctgagagtgaacaccgagatcaccaaggcccccctgagcgcctctatgatcaagagatacgacgagcaccaccaggacctgaccctgctgaaagctctcgtgcggcagcagctgcctgagaagtacaaagagattttcttcgaccagagcaagaacggctacgccggctacattgacggcggagccagccaggaagagttctacaagttcatcaagcccatcctggaaaagatggacggcaccgaggaactgctcgtgaagctgaacagagaggacctgctgcggaagcagcggaccttcgacaacggcagcatcccccaccagatccacctgggagagctgcacgccattctgcggcggcaggaagatttttacccattcctgaaggacaaccgggaaaagatcgagaagatcctgaccttccgcatcccctactacgtgggccctctggccaggggaaacagcagattcgcctggatgaccagaaagagcgaggaaaccatcaccccctggaacttcgaggaagtggtggacaagggcgcttccgcccagagcttcatcgagcggatgaccaacttcgataagaacctgcccaacgagaaggtgctgcccaagcacagcctgctgtacgagtacttcaccgtgtataacgagctgaccaaagtgaaatacgtgaccgagggaatgagaaagcccgccttcctgagcggcgagcagaaaaaggccatcgtggacctgctgttcaagaccaaccggaaagtgaccgtgaagcagctgaaagaggactacttcaagaaaatcgagtgcttcgactccgtggaaatctccggcgtggaagatcggttcaacgcctccctgggcacataccacgatctgctgaaaattatcaaggacaaggacttcctggacaatgaggaaaacgaggacattctggaagatatcgtgctgaccctgacactgtttgaggacagagagatgatcgaggaacggctgaaaacctatgcccacctgttcgacgacaaagtgatgaagcagctgaagcggcggagatacaccggctggggcaggctgagccggaagctgatcaacggcatccgggacaagcagtccggcaagacaatcctggatttcctgaagtccgacggcttcgccaacagaaacttcatgcagctgatccacgacgacagcctgacctttaaagaggacatccagaaagcccaggtgtccggccagggcgatagcctgcacgagcacattgccaatctggccggcagccccgccattaagaagggcatcctgcagacagtgaaggtggtggacgagctcgtgaaagtgatgggccggcacaagcccgagaacatcgtgatcgaaatggccagagagaaccagaccacccagaagggacagaagaacagccgcgagagaatgaagcggatcgaagagggcatcaaagagctgggcagccagatcctgaaagaacaccccgtggaaaacacccagctgcagaacgagaagctgtacctgtactacctgcagaatgggcgggatatgtacgtggaccaggaactggacatcaaccggctgtccgactacgatgtggaccatatcgtgcctcagagctttctgaaggacgactccatcgacaacaaggtgctgaccagaagcgacaagaaccggggcaagagcgacaacgtgccctccgaagaggtcgtgaagaagatgaagaactactggcggcagctgctgaacgccaagctgattacccagagaaagttcgacaatctgaccaaggccgagagaggcggcctgagcgaactggataaggccggcttcatcaagagacagctggtggaaacccggcagatcacaaagcacgtggcacagatcctggactcccggatgaacactaagtacgacgagaatgacaagctgatccgggaagtgaaagtgatcaccctgaagtccaagctggtgtccgatttccggaaggatttccagttttacaaagtgcgcgagatcaacaactaccaccacgcccacgacgcctacctgaacgccgtcgtgggaaccgccctgatcaaaaagtaccctaagctggaaagcgagttcgtgtacggcgactacaaggtgtacgacgtgcggaagatgatcgccaagagcgagcaggaaatcggcaaggctaccgccaagtacttcttctacagcaacatcatgaactttttcaagaccgagattaccctggccaacggcgagatccggaagcggcctctgatcgagacaaacggcgaaaccggggagatcgtgtgggataagggccgggattttgccaccgtgcggaaagtgctgagcatgccccaagtgaatatcgtgaaaaagaccgaggtgcagacaggcggcttcagcaaagagtctatcctgcccaagaggaacagcgataagctgatcgccagaaagaaggactgggaccctaagaagtacggcggcttcgacagccccaccgtggcctattctgtgctggtggtggccaaagtggaaaagggcaagtccaagaaactgaagagtgtgaaagagctgctggggatcaccatcatggaaagaagcagcttcgagaagaatcccatcgactttctggaagccaagggctacaaagaagtgaaaaaggacctgatcatcaagctgcctaagtactccctgttcgagctggaaaacggccggaagagaatgctggcctctgccggcgaactgcagaagggaaacgaactggccctgccctccaaatatgtgaacttcctgtacctggccagccactatgagaagctgaagggctcccccgaggataatgagcagaaacagctgtttgtggaacagcacaagcactacctggacgagatcatcgagcagatcagcgagttctccaagagagtgatcctggccgacgctaatctggacaaagtgctgtccgcctacaacaagcaccgggataagcccatcagagagcaggccgagaatatcatccacctgtttaccctgaccaatctgggagcccctgccgccttcaagtactttgacaccaccatcgaccggaagaggtacaccagcaccaaagaggtgctggacgccaccctgatccaccagagcatcaccggcctgtacgagacacggatcgacctgtctcagctgggaggtgactctggcggctcaaaaagaaccgccgacggcagcgaattcgagcccaagaagaagaggaaagtctaa

SEQ ID NO: 202 - DNA, 35 bp, synthetic construct
  source 1..35: mol_type = other DNA
gaagcggaaagtcgacaagaagtacagcatcggcc

SEQ ID NO: 203 - DNA, 39 bp, synthetic construct
  source 1..39: mol_type = other DNA
ctgtacttcttgtcgactttccgcttcttctttggtgac

SEQ ID NO: 204 - DNA, 119 bp, synthetic construct
  source 1..119: mol_type = other DNA
tctggaggatctagcggcggatcctctggaagcgagacaccaggcacaagcgagtccgccacaccagagagctccggcggctcctccggaggatccggaatgagtgagctgaatgatgc

SEQ ID NO: 205 - DNA, 40 bp, synthetic construct
  source 1..40: mol_type = other DNA
tgaccccccgctgctgcccccgctgctttcaggtgttgcg

SEQ ID NO: 206 - DNA, 44 bp, synthetic construct
  source 1..44: mol_type = other DNA
ggggcagcagcggggggtcagtggaagatcggttcaacgcctcc

SEQ ID NO: 207 - DNA, 45 bp, synthetic construct
  source 1..45: mol_type = other DNA
ccgccgctagatcctccagagccggagatttccacggagtcgaag

SEQ ID NO: 208 - DNA, 49 bp, synthetic construct
  source 1..49: mol_type = other DNA
ggggcagcagcggggggtcacagaccacccagaagggacagaagaacag

SEQ ID NO: 209 - DNA, 54 bp, synthetic construct
  source 1..54: mol_type = other DNA
ccgccgctagatcctccagagttctctctggccatttcgatcacgatgttctcg

SEQ ID NO: 210 - DNA, 46 bp, synthetic construct
  source 1..46: mol_type = other DNA
ggggcagcagcggggggtcaacccagaagggacagaagaacagccg

SEQ ID NO: 211 - DNA, 51 bp, synthetic construct
  source 1..51: mol_type = other DNA
ccgccgctagatcctccagaggtctggttctctctggccatttcgatcacg

SEQ ID NO: 212 - DNA, 43 bp, synthetic construct
  source 1..43: mol_type = other DNA
ggggcagcagcggggggtcaaacagccgcgagagaatgaagcg

SEQ ID NO: 213 - DNA, 45 bp, synthetic construct
  source 1..45: mol_type = other DNA
ccgccgctagatcctccagacttctgtcccttctgggtggtctgg

SEQ ID NO: 214 - DNA, 42 bp, synthetic construct
  source 1..42: mol_type = other DNA
ggggcagcagcggggggtcaagccagatcctgaaagaacacc

SEQ ID NO: 215 - DNA, 49 bp, synthetic construct
  source 1..49: mol_type = other DNA
ccgccgctagatcctccagagcccagctctttgatgccctcttcgatcc

SEQ ID NO: 216 - DNA, 45 bp, synthetic construct
  source 1..45: mol_type = other DNA
ggggcagcagcggggggtcaagaggcggcctgagcgaactggata

SEQ ID NO: 217 - DNA, 54 bp, synthetic construct
  source 1..54: mol_type = other DNA
ccgccgctagatcctccagactcggccttggtcagattgtcgaactttctctgg

SEQ ID NO: 218 - DNA, 48 bp, synthetic construct
  source 1..48: mol_type = other DNA
ggggcagcagcggggggtcaagacagctggtggaaacccggcagatca

SEQ ID NO: 219 - DNA, 48 bp, synthetic construct
  source 1..48: mol_type = other DNA
ccgccgctagatcctccagacttgatgaagccggccttatccagttcg

SEQ ID NO: 220 - DNA, 40 bp, synthetic construct
  source 1..40: mol_type = other DNA
ggggcagcagcggggggtcagagacaaacggcgaaaccgg

SEQ ID NO: 221 - DNA, 63 bp, synthetic construct
  source 1..63: mol_type = other DNA
ccgccgctagatcctccagacttgaaaaagttcatgatgttgctgtagaagaagtacttggcg

SEQ ID NO: 222 - DNA, 43 bp, synthetic construct
  source 1..43: mol_type = other DNA
ggggcagcagcggggggtcaatcgagacaaacggcgaaaccgg

SEQ ID NO: 223 - DNA, 65 bp, synthetic construct
  source 1..65: mol_type = other DNA
ccgccgctagatcctccagaggtcttgaaaaagttcatgatgttgctgtagaagaagtacttggc

SEQ ID NO: 224 - DNA, 48 bp, synthetic construct
  source 1..48: mol_type = other DNA
ggggcagcagcggggggtcacccgaggataatgagcagaaacagctgt

SEQ ID NO: 225 - DNA, 47 bp, synthetic construct
  source 1..47: mol_type = other DNA
ccgccgctagatcctccagaggagcccttcagcttctcatagtggct

SEQ ID NO: 226 - DNA, 48 bp, synthetic construct
  source 1..48: mol_type = other DNA
ggggcagcagcggggggtcaaagcactacctggacgagatcatcgagc

SEQ ID NO: 227 - DNA, 48 bp, synthetic construct
  source 1..48: mol_type = other DNA
ccgccgctagatcctccagagtgctgttccacaaacagctgtttctgc

SEQ ID NO: 228 - DNA, 47 bp, synthetic construct
  source 1..47: mol_type = other DNA
ggggcagcagcggggggtcattctccaagagagtgatcctggccgac

SEQ ID NO: 229 - DNA, 50 bp, synthetic construct
  source 1..50: mol_type = other DNA
ccgccgctagatcctccagactcgctgatctgctcgatgatctcgtccag

SEQ ID NO: 230 - protein, 1629 aa, synthetic construct
PKKKRKVMDKKYSIGLAIGTNSVGWAVITDEYKVPSKKFKVLGNTDRHSIKKNLIGALLFDSGETAEATRLKRTARRRYTRRKNRICYLQEIFSNEMAKVDDSFFHRLEESFLVEEDKKHERHPIFGNIVDEVAYHEKYPTIYHLRKKLVDSTDKADLRLIYLALAHMIKFRGHFLIEGDLNPDNSDVDKLFIQLVQTYNQLFEENPINASGVDAKAILSARLSKSRRLENLIAQLPGEKKNGLFGNLIALSLGLTPNFKSNFDLAEDAKLQLSKDTYDDDLDNLLAQIGDQYADLFLAAKNLSDAILLSDILRVNTEITKAPLSASMIKRYDEHHQDLTLLKALVRQQLPEKYKEIFFDQSKNGYAGYIDGGASQEEFYKFIKPILEKMDGTEELLVKLNREDLLRKQRTFDNGSIPHQIHLGELHAILRRQEDFYPFLKDNREKIEKILTFRIPYYVGPLARGNSRFAWMTRKSEETITPWNFEEVVDKGASAQSFIERMTNFDKNLPNEKVLPKHSLLYEYFTVYNELTKVKYVTEGMRKPAFLSGEQKKAIVDLLFKTNRKVTVKQLKEDYFKKIECFDSVEISGVEDRFNASLGTYHDLLKIIKDKDFLDNEENEDILEDIVLTLTLFEDREMIEERLKTYAHLFDDKVMKQLKRRRYTGWGRLSRKLINGIRDKQSGKTILDFLKSDGFANRNFMQLIHDDSLTFKEDIQKAQVSGQGDSLHEHIANLAGSPAIKKGILQTVKVVDELVKVMGRHKPENIVIEMARENQTTQKGQKNSRERMKRIEEGIKELGSQILKEHPVENTQLQNEKLYLYYLQNGRDMYVDQELDINRLSDYDVDHIVPQSFLKDDSIDNKVLTRSDKNRGKSDNVPSEEVVKKMKNYWRQLLNAKLITQRKFDNLTKAERGGLSELDKAGFIKRQLVETRQITKHVAQILDSRMNTKYDENDKLIREVKVITLKSKLVSDFRKDFQFYKVREINNYHHAHDAYLNAVVGTALIKKYPKLESEFVYGDYKVYDVRKMIAKSEQEIGKATAKYFFYSNIMNFFKTEITLANGEIRKRPLIETNGETGEIVWDKGRDFATVRKVLSMPQVNIVKKTEVQTGGFSKESILPKRNSDKLIARKKDWDPKKYGGFDSPTVAYSVLVVAKVEKGKSKKLKSVKELLGITIMERSSFEKNPIDFLEAKGYKEVKKDLIIKLPKYSLFELENGRKRMLASAGELQKGNELALPSKYVNFLYLASHYEKLKGSSGGSSGGSSGSETPGTSESATPESSGGSSGGSSELNDAYWMKQALALAQKAREQGEVPVGAILVLDDEVIGQGWNRAITLHDPTAHAEIMALQQGGQIVQNYRLLNATLYVTFEPCVMCAGAMVHSRIKRLVYGVSNSKRGAAGSLLNVLNYPGMNHQIEITAGVMANECSEMLCQFYQQPREVFNAEREARRLNQPDRADSGGSSGGSSGSETPGTSESATPESSGGSSGGSPEDNEQKQLFVEQHKHYLDEIIEQISEFSKRVILADANLDKVLSAYNKHRDKPIREQAENIIHLFTLTNLGAPAAFKYFDTTIDRKRYTSTKEVLDATLIHQSITGLYETRIDLSQLGGDSGGSKRTADGSEFEPKKKRKV

SEQ ID NO: 231 - RNA, 20 nt, synthetic construct
  source 1..20: mol_type = other RNA
ggaacacggataaagacgct

SEQ ID NO: 232 - DNA, 19 bp, synthetic construct
  source 1..19: mol_type = other DNA
atggatgtggcgcaggtag

SEQ ID NO: 233 - DNA, 19 bp, synthetic construct
  source 1..19: mol_type = other DNA
aaggaagcgcggagacgtt